European Patent Application EP 4 368 186 A1, published May 15, 2024. Title: Agent for reducing nephrotoxicity. Applicant: NIPPON SHINYAKU CO., LTD. Application JP. The sequence listing filed with the application follows.

SEQUENCE LISTING (13 sequences)

SEQ ID NO: 1 - DNA, 22 bp, synthetic construct
  misc_feature 1..22: note = Synthetic
  source 1..22: mol_type = other DNA
gctcggcatcagagggagaccg

SEQ ID NO: 2 - DNA, 20 bp, synthetic construct
  misc_feature 1..20: note = Synthetic
  source 1..20: mol_type = other DNA
ctcggcatcagagggagacc

SEQ ID NO: 3 - DNA, 17 bp, synthetic construct
  misc_feature 1..17: note = Synthetic
  source 1..17: mol_type = other DNA
cggcatcagagggagac

SEQ ID NO: 4 - DNA, 20 bp, synthetic construct
  misc_feature 1..20: note = Synthetic
  source 1..20: mol_type = other DNA
ccttggctcggcatcagagg

SEQ ID NO: 5 - DNA, 21 bp, synthetic construct
  misc_feature 1..21: note = Synthetic
  source 1..21: mol_type = other DNA
catcagagggagaccgtgtaa

SEQ ID NO: 6 - DNA, 21 bp, synthetic construct
  misc_feature 1..21: note = Synthetic
  source 1..21: mol_type = other DNA
ctcgtgcatcagagggagacc

SEQ ID NO: 7 - DNA, 19 bp, synthetic construct
  misc_feature 1..19: note = Synthetic
  source 1..19: mol_type = other DNA
ctcgcatcagagggagacc

SEQ ID NO: 8 - DNA, 25 bp, synthetic construct
  misc_feature 1..25: note = Synthetic
  source 1..25: mol_type = other DNA
aggagggcagcgaactcctggttgt

SEQ ID NO: 9 - DNA, 25 bp, synthetic construct
  misc_feature 1..25: note = Synthetic
  source 1..25: mol_type = other DNA
gtggttgagccagaagctgggaatt

SEQ ID NO: 10 - DNA, 25 bp, synthetic construct
  misc_feature 1..25: note = Synthetic
  source 1..25: mol_type = other DNA
gttgcctccggttctgaaggtgttc

SEQ ID NO: 11 - DNA, 22 bp, synthetic construct
  misc_feature 1..22: note = Synthetic
  source 1..22: mol_type = other DNA
caatgccatcctggagttcctg

SEQ ID NO: 12 - DNA, 21 bp, synthetic construct
  misc_feature 1..21: note = Synthetic
  source 1..21: mol_type = other DNA
cctccggttctgaaggtgttc

SEQ ID NO: 13 - DNA, 134937 bp, Homo sapiens
  source 1..134937: mol_type = genomic DNA
gatctttggtttgctttcccaacttatattgtgaactgccttctcttcatcccaacattcctgatgttgctgtgtctcagtttacagatgttaaggaacttataatcaaaactgtattaagctcggcaagagatgagccctctggtcctgcacgatgtgtagcactttgtagtttaggtatttggatttgtgaagaactagtccatgagtctcatcatcctcaaattaaggaagctctgaatgtgatttgtgtttccttaaagtttactaataaaacagtagcccacgtagcttgtaacatgcttcacatgctggttcattatgtacctagacttcagatttaccagcctgattctcccttgaaaattattcagatcctaatagctaccatcacccatcttttaccaagtacagaggcttcatcttatgaaatggacaagaggttggtagtatctttacttctctgccttctggactggatcatggccttacctctaaagacactgctccaaccatttcatgctacgggagcagaaagcgataaaacagaaaaatctgttctcaattgcatttataaggttttacatgggtgtgtttatggagctcagtgttttagcaatccaaggtattttcccatgagcctctctgatttggcatctgtagattatgatccttttatgcatttggaaagtctgaaagagcctgagcctctgcgctctcctgactcagaacgatcttctaaactccagccagtaacagaagtgaaaactcaaatgcagcatggattaatctctatagcagcccgcactgttattacacatctggtaaatcacctgggccattatccaatgagcggtggtcctgctatgctaacaagtcaggtgtgtgaaaatcacgacaatcattacagtgaaagtactgaactttctcctgaactctttgagagtccaaatatccagttctttgtgttaataatacaaccttagtgtcctgtatccagatcagatcagaagagaatatgcctggaggaggtttatctgctggccttgcatcagccaattcaaatgtcagaatcatagtacgtgatctctctggaaaatattcatgggattctgctatactgtatggcccacctcctgtaagtggcttgtcagaacctacatctttcatgctttcattgtctcaccaagagaagccagaagagcctccgacatctaatgaatgcttagaagatataaccgtaaaagatggactttccagtttaaaagatttagagaaactgtaccaacttgggatacaataagagatgaagaagatgctcttgatgaactcttgcagtatttgggtgttactagtcctgaatgcttacagagaactggaatctcacttaatattcctgctccacaacctgtgtgcatttctgaaaaacaagaaagtgatgttattaatgctatccttaagcaacatacagaagaaaaagaatttgttgagaagcactttaatgacttaaacatgaaagctgtggaacaagatgaaccaatacctcaaaaacctcagtcagcattttattattgcagattgcttcttagtatattgggaatgaattcctgggacaaacggaggagctttcatctcctgaagaaaaatgaaaagctacttagagaacttaggaacttggattcaaggcagtgccgagagacacacaagattgcagtattttatgttgctgaaggacaagaagacaaacactccattctcaccaatacaggaggaagtcaagcatatgaagattttgtagctggtcttggttgggaggtaaatcttacaaaccattgtggttttatgggaggactacaaaaaaacaaaagcactggattgaccactccatattttgctacctctacagtagaagtaatatttcacatgtcaacaagaatgccttctgattctgatgattctttgaccaaaaaattgagacatttgggaaatgatgaagtgcacattgtttggtcagagcatactagagactacaggagaggaattattcccacagaatttggtgatgtccttattgtaatatatccaatgaaaaatcacatgttcagtattcagataatgagaaaaccagaggttcccttctttggtcccctttttgatggtgctattgtgaatggaaaggttctacccattatggttagagcaacagctataaatgcaagccgtgctctgaaatctctgattccattgtatcaaaacttctatgaggagagagcacgatacctgcaaacaattgtccagcaccacttagaaccaacaacatttgaagattttgcagcacaggttttttctccagctccctaccaccatttaccatctgatgccgatcattaaatatcagttctgtttatctgaaggctcctacccagagattctacccagtgaaactcccacagcagcgcaggtagatggggctgacctggcctctccaatgtctcctcgaactagcaaaagccgcatgtccatgaagctgcgtcgttcctctggctcagccaataaatcctaaggagacaagcagcccagcagtgatcagcagtagccaccttagcatgaacatagggttaaccctttcaggccttcatgtctgccataacatgcatgtttcttcctgtacatttatttgagaaaacactggatttaaataattttaaataatttgtagcttaatattaaagatttaagttatttattgtttcatttttttcccacaatccaagctgccatattttgagggcagggggagttttattctacaccctttaccttcctagataattatgtctaagtagttttatctttaatttcatggttaactgtgagccaaaatacaattggacaattagtctcattatttattgtgctccattgcaactttatggttcaataaatatataattttttacaaatgtaaaattttacatttaagcatttgtaaagttacagcaaaagatgtacctgttaatacacagaatgtgtacagattatttgttatgacaataaaacactcaaaataaatggtctttagcatctcaaattccaactgaaatcattttagtattaactcttcttcccaaagcaatgtctcatttcttggctgtgcaggtgatgccatgttatatccaataactagaaaaatcactgtgctgaacttttatgtttagcttccaagtatttttctaatgttttgcatttcaagtggtatcactgttaaatgccatttgttttcagattgtggccttttattattggctgctagatcctggtgtttctatgttcttttttaagcaccaaaaagaagatggggaagaaaagaaggaaaattttctgatataaatatgttgttcaaattatgagtactatttaaaaaagaaaaaggaacctaacccaggagtctaagttaaatctaatattgttaatactgaacttgcaggtccaggttggtatacattccaccctctagaagtattttcttacagtagataagctgctcacattttgttttgaatgggcatctcctgaggaaatgtagcatgatattggtactaactgcatgtgtaaatacatcatactggcaagccgtaaaatataaattatgtatcattcacgtagtatctataatttgtaacagtggggggaaaagatgacatggtatttaataatacaataaaaatattcttatcaaaaaaaaaaaagaaaagaaaaccagcacaagacaaggatgccctctctcaccactcctactcaacatagtattgaaagttctgaccagggcaatcaggcaagagaaagaaataaagcgtattcaaataggaagagaggaagtcaaattgtctctgtttgcagatgacatgattgtatatttagaaaaccccatcttttcagcccaaaatctccttaagcttataagcaacttcagcaaagtctcaggatacaaaatcaatatgcaaaaatcacaaacattcctataccccaatgacaggcaaacagagagccaaatcatgagtgaactcttattcacaattgctacaaagagaatacgtaggaatacaacttacaagggatgtgaaggacatcttcaaggagaactacaaaccactactcaaggaaataagggaggacacaaacaaatggaaaaacattccatgctcatggataggaataatcaatatcgtgaaaatggccatactgctcaaagtaatttatagattcaacgctattcccatcaagctaccattgactttcttcacagaattggaaaaagctactttaaacttcatatggaaccgcccgcatagagaagacaatcttaagcaaaaagaacaaagctagaggcatcatgctacctgacttcaaactatactacaaggctacagtaaccaaaacagcatggcactggtaccaaaacagatacatagaccaatggaagagaacagagacctaagaaataaaaccacacatctacaaccatctcatctttgacaaacctgacacaaacaagcaatggggaaaagattccctatttaataaatggtgttgggagaactggctagctatgcagaaaactgaaactggaccccttccttacaccttacacaaaaatcaactcaagatggattaaagacttaaagataagacctaaaaccataaaaatcctggaagaaatcctaggcaataccattcaggacataagcatgggcaaagacttcatgtctaaaataccaaaagcaatggcaacaaaagccagaattgacaaatggaatctaattaaactaaagagcttctgcacagcaaaagaaactgtcatcagagtgaacaggcaacctacagaatgggagaaaatttttgcaatctatccatctgacaaagggctaatatccagaatctacaaagaacttaaccaaatttacaagaaaaaaacaaccccatcgaacagtgggcaaaggatatgaacagacacttatcaaacatatgctaacaaagatattaaaaaaaatgctcatcatcactggtcattagagaaatgcaaatcaaaaccaccatgagataccatctcacgccagttagaatggcgatcatgaaaaagtcaggaaacaacagatgctggagaggatgtggagaaataggaactgttctacactgttggtgggagtgtaaattaattagttcaaccattgttgaagacagtgtggcgattcctcaaggatctagaactagaaatatcatttgacccagcaatcccattactgggtatatacccaaaggatttataaatccttctactataaagtcacatgcacacatatgtttatcgggtcactattcacaacagaaagccttggaaccaattcagatgtccatcaatgatagactggataaagaaaatgtggcacatatacaccatggaatactacacagccataaaaaaggatgagttcatgtcctttgcagggacactgatgaagctggaaaccatcattctcagaaactatgacaagaacagaaaaccaaacgccacgtgttctcactcataagtgggagttgaacaatgagaacgcgtggacacagagaggggaacatcacacatggggcctgtcggggtgggggtctagaggtggaatagcattaggagaaattcctaaggtaggtgaccggttgatgagtgcagcaaaccaccatgacacatgtatacctatgtaacaaaactgcacattctgcacatgtaccccagaactttaagtataataatattaaaaaaaaaagagaaaaaaaatcacacacaggatttgggtctggagcaagagtcctgagacaggttatttaacctgttagaatttgggggactttcattaaagaagtggtatttaggccggttcttgagcaagtgggaaaatgtatggttgttagacttgcagtgaaaggcggaacagccatagcaaaggcactgaagcagatggtgtgagtttaaacaacattttgactggtatatttagctatatagtgctctctaggagttagaaggctagaaaggcagattaggactaaatcaagaaccagaatgtcatgctaagtcgtttgtaagtagtatagaagtaaatgatgatttttaaatagaggaatcagagtaagctttatcttgtaataatgaaaaagatgaattggacagtaaagaaattatctgggaagctggtaaaacagtccagactagaggtagctgaagaggcttacttaaattcagatagttaagtggccagggtgtcctttagggaagtggggtgagggaggggatgggaggagatcatgcttgacataaaacttattataagttgtttcttgcaaaagtgacttaggattggaagtctggaatgctgcaatggaagagttttccttacttaacttttctctgaaattaaactgccaatgtcaatagttatgtctgtttttcttttctccatgcttccctttatttctttactactggtaagttacaaatttttaaaaattgtttttctgttatcaaaagagctcttaatacattttgaagcagtgctaagtgaaatttttctctttatttgtatgacgttcactttctatttgttgccctgagttacttgggaaatatttttcagaatgcatgtttcctctcagcagacactctgaccaccagttggggaggcaaactatcagtgtattttgaaaaagtttcctgattgtttctgaatctgctgtgccttttcaattgacaatcattgatttattacaaaatgccaaaggcctttgttttttcaatttagtactttggctcaggaagatacaggtgttccttaattgatagtatcacatactctactcagctgagctcattctagtcagatattgtacacctactctgtactgaggatacagagatgagatgtggatcctagcaacagttagttcccttccctcagctactccatagccaagttcctcacttgccgtaaccaataagcgctaagcatgccgtatgatagatttgtaaaacctgtcttttcatcacccttttaatccctactccttgatagaggagttttgctttgttttacctcagtggctcctagcccagatgaacagcaaaatcctgaaattcttaatttaaaaaccagacatgtgtttctcaagcctaccctccagtatctgatttagtagtttatggtaagtcctggtaatttgcatttttaaaaggtccccaagtgattctgatgtgcagctgggttgaagaaccactggtttggttcatttaattcctcctcactcctgattacacatttactttaacctctcctctcctttcatttcattcttacctagttacccaaaacaaaatcttgttgactttctttgctctgtttcttagctgaatagcaaccatagtcatgattgttaatggtaagatagtactagcaatactaaaaagcactggggcttaaagtgaagttagatataatgaagagctagtgttctcaggttattgtatcccatcttccttctctagttacaaaagtaatttttacaaatactgacgtgattaattaaaactgtgttcatttttgtatagttaccaatatttgctgttgaataacttgggtggaggaagattaatgtgcagtcaatttatgaattggtgacttgatgaattgggtaatatttggtgacctctgcactcattttttctaggggagaatgtactttcatttcagataatgtcacatgaacttttggagaataactgtcaaccacaggaagttcttttattatataggtgttctggagacctaaaagcttttttgttataatttatataccgtgttgaaacaattttactttcgccctcttccttttcatgtcttcttttaatgttgcatctaaaacattgttttttcacacctctttttaagaaaagcaacagcatggtttctttcatgaaatgtttccagaagcctgatccaaaaagagaaaagtatagctggttaaaggagggaggaagccctaaatctggcttcttcccagagtacctctgtggcatctgtggattcccttgagttcagcacatggtttaaacaccattgatttcaagagtctttgcccctcacaagatcaggaaaatagagctgcatgtactatttttttaaactttgaggcaaatgtaatgttatcttttctcctgagcttaagataaagcttttgaaaacatacagaccttttgtgatcgggcttttaacattctctatcagcttgtataaaatgaatcagaaagaaaattatgatacagttcttttttcctgagttatcagttgacaatgtttgcagttttactttcttactatactagttaatgactcttacaagtattgtataagatcagcttagaatacatgttcatctcaaaccttgaagaagtgaaaacatatatttttggtattcagaataaaaagtataaatgtttaataatttttatttgtttctatccttcattttggagatctcaacaactattctggaattttcccccctcacgttctgttttgctgtccccgtacccaatagcaagaaactactgcctaccttagcacaagtttcacagaaattttaatctacctatccacattcagctttgctcatgctatctgttcaaacagaacttatagtcagtttttagttgtctttttaaagaaacatctttacacaaaggacctttgaaatcccttgggaagaattaaactaagtcatgtgagtgttgtagttctagacttacacttttgctacttaatattatacactaaaaaggagacagttgaagtggtcctgagttctttgaaattgtctaataagtctgatttctgacagcaagacatttaaataatgcagaatgaagtcactgaatcatatgaaatgaatcatatgaaatgactttaagttttatctgtattcttgctttgccatcagggatttctagtctagtattggtagcttatattaaaatctactcagttgatcttttcttaggaagaaaatttctagtgctatgttagaaaaaagtgtttttatttctaactagtggtgagaatatagttatccccatatcccccaaatacttttaggataatcttgaccaaaaaatcttttgttaaatgcagtaattcaatataattaaaatgtttttgaaaacatctttgggactgaatctgttttgagtttttgaatgttagtaaacatcccaatactccagttttccatatatcatataatttgatataagaggaagtcaaggtggatcttgtctatttgagtaggagaaatgcttgataatacttgatattatcctgtgcaaggatttggataattgccatttccatcttttttttttttttttgagatggcgtctagccctgttgcccaggctggagtgcagtggcgccatctcggctcactacaacctctgcttcctgggttcaggcaattctcctgcctcagcctcccgagtagctgggattacaggcacccacaaccacacccagctaatttttgtatttttagtagaaacggggtttcactgtgttgcccaggctggtctcgaactccagacttcgagatccacctgtcttggcctctcaaattgctgagattagaagcatgagccaccgcgtgcagccccccgtccctttttttttaagacagagttttgctcttgttgcctaggctggagtgcaatggtgcaatcatggctcacccgcaacctctgactcctgggttcaagcgattctcctgcctcagcctcccgagtagctgggattacaggcatgtgccaccacgccctactaattttgtatttttagtagagatggggtttctccacgttagtcaggctcgtctcgaactcccgacctcaggtgatcctcctgccttggcgcctcccaaagtgctgggattacaggtgtgagccaccgtgcctggccgccatttctatttttaagaaggtaagattcagagcaaaaatactcactgcttataaaaagagttatttagtcaggattataagaagaaacctatttttgccttcatttaactgcaaaaaaatgtaagctgtaactcattatctttcttgagttcttttttttctttagtaaatcttgtcacattttagcattgtttcttatttcagccgtgtattctttgtataagccttgctcagtctgcatgccattagtgttttcagcctgctttgtattgatagcttcttacatttcagtgtttataattgacagcgctctttaattaactagttcagatcaaattgaatggtgttatttctataacataattagaaatcttttcagaggttccttccatgatttctagttttagtttatgaaacatttacagtataaaatatttgtttttcttttttctttttgtttatatagaagtggtacaccatccccaaaacgaacatctgtaggctccaggccaccagcagtaagaggcagtagagatcgttttactggagaatcatacacagtgctgggtaggacaaaacataattgtttttcattatctcagattaaaggcatcacaatcacactggtggactttccactcaaagtgactgcctgtatattgaataaatctttgcaagaaatttctcccaattgaagcctaattactttggggagttttcagattgtcttattattattgatacttttaaaactctacttcagcttacgtagtgttcccacatctttatatataagccgggaggggggatagtaaggaagaaaacctctgaagcgttttatattcaagaatagtactaaacgtaaaggtaaagttagagcaggtactcagcatttaatgtctgtgtgttaacatgattattcttataggaaaagtacttgaataaaaatttttgtgtctttttttgggacgagtggtaggtaaaactgtgtgactcataaggaagagatgagtcaaatctacctttctgatcttttgtaggagacactgctattgaaagtggacaacattattgggaggtcaaggcccagaaggattgtaaatcctacagtgtgggagtagcatacaaaacgttggggaaatttgaccaattgggaaagacaaacactagttggtgtatccatgtcaacaactggctacaaaacacatttgcagcaaagcataataataaagtcaaagctttggatgttactgttcctgaaaaaataggtgtattttgtgattttgatgggggtaagtttattttctcgtaggttatttcatcatagttgcttgcatttcagtacctttcactggtaatcatctatacaggatttccattagtattgtgggaaggacattttgatcaggtaggcttttgattgcaatcataatctcaattctagaattgactggaatggtatatgtgatgtctgcctggagccctataaaagcactcatttataatatactaagtctgaaagattttgctaattttagtcttcagcactaacatttcttctgtccattttaattccttccttaccatgttttattacctacctctaaagagtgatagtcaaaattttctagttgaagtagatcttagaaattacccaacccaggatgaataccccattttacatgatgtgattattacacattgcatgcctatatgaaagcatctcatatactgcgtaaacatacacacctactatgtacctacaaaaattaaaaaaaaattcaagaagataccagagccatattttctactatcctagtaaacataagctatacagcaaatatttactgtgccaaaccgcatcacacttgaaacaaatggaatgttcttaattttcaagttgctgtctttaaaaatattcttcagaatgactcatgatatctttagaggggccaaaggggtttcccctcaatatcagaatttctttacttacaaaattattaacacagtgtagtctaatccaaaaaagaaaagaaattactccatctgccacacagtatacagttcttagtacactatctctgcaggtagttgccacttatgtgcctgaagaacttttaatgtgaagtttactgtcttagaaagcagcctgtttcattgttggacagctcttggttagaagatttttcttaagttgactcacattgtttcccttaaattttcccatctgaataaacacagaattacgtttcctcactcatgttcacacgataatcctttattaaaaactttcttgccctgtttttccagaccatatattctgttattagctgcccctgttaaaatttaatttttccaagtctttataatctcctatggctgtctagtatgtcagtgtttttcttaaaggttggtcttagagtggaacacatgacctctgaccagcaaaggacagtaatttggctatgctatttctaatagtatgacttagcactgctgatcaatattgagcttgtagctaccctaatccattagatcttttttcacggcattatgtcaaattgtctttttcttttgttaggcagtttatggttttggttttttttgttttgttttgttttgtttttgagacagagtcttactctgttgtccaggctggagtgcagtggctcaatctcagctcactgcaacctctgcctcccatgttcaagcgactctcctgcctcagcctcctgagttagctgggattacaggtgcatgccaccacgcctggctaatttttgtatttttagtagagacggggtttcaccatgctggccaggctggtctcaaactcctgacctcaagtgatccacctggctgggcctcccaaagtgcagggattactgccatgagccaccacacccagccagtttatggtttttaaaaataactcaatgttatatgtaatgcaaatgaagactattacatttacccttttttagtttcatcttaatagatttggcccaaatttcccgtcttaaaattatctaaaaatttacttgatatttatattttgaaaaaattttaaagctcattgaattagttatttcataagcatattctctacagtcatctaatgtataataattttgaagatgacataatattgaactaaagtaattccctagatgttttttctccaagttgacacttaagctaataccaaattttattattttagtaatattgtgcccaaataattccatgagctgtcagttaatttactcaaaaaaggagaaaaagtaattttggcttgatttatttttagtgatgacatgttagctttgctgtgttttttgttttttaacttattcaccttgaatcagttaaatcattttcctcaggataaatggcaaatttattagcacacatttttttttcaactaccaagacaacatttgcttcttctctctcctttcccatactctgtgagtccataaaggtagtagtgagatacagtttttagtctagaacataacgtatggcaaggggaagttgtactgtggaataggatcagattctgagagccttgaaaaataataatggactggtcttcagtagtggggaggggtggttctgcatgttttagaacactatagtcataagataattgagttttagaaatattagagagtcagtggttaaagatggaagagatcgaaagcatagcaagcataagacttttcgggaagcagtcttcaagtggtgtagagcaggactgagtctcttgttagctattaagcccttattgcctggctagtgcttttcacatagaaagcccttaataagtgttgagtaactggcaacaagcatctgagcagtggagaattaagaatggatttgacagtgtagaagtagaattcataggacttagtaactaaatacagatcagctgaggacagacagttgaagatgactttgaggttccagccagtgtgatcaagaggatgacagtgtcaacaggatagggaacatagagttttggggggaaatgaaatgccagcaggataatcatgtggcatgtttagcaagcattttgaaattcagtgctagaattcagcagttaagtagagctgacattaaatatttgagacagcattacagaattgctatggaagattgtacaggacaatatatttaagcattactattctgctgtttactaactttgtgatcatatgtaccgttatgctgtttaccaacttcgagatcaaagtactgggtactttacatacattacctcaaaatattaaacaatctacataataatgtgcataaatattagtttattttatcttcctctttggtggcagttgatttattaaggaagcattatataaagaaaagagagcatggacaaagtggctacatttagaacaggaagaaaaggaggagatggtgaagttatccccagggttatgatacaaaccaagggaatggtcatcagagaagagtttcaagaagtgataacagctgtaaggaggccatttggttggccagtttaggaggtcagacagacagttttttttagggcatgatcctattgaaggatatactgtgaggtgattttaaaaattaacaaagcaggtcaggcatagtggctcatgcttgtaatcctagcactttgggagactgaggtggaggattgcttgagctcaggagttcaagcccagcttatacaaaatagcaagaccccgcctctgttaaaaaaattaacaaaattgaagcagtgatagatatattgtgattttagagactggagtatcagtatcgcatcaggtagatagaagacaaggtttaatagagtaaaccttaaatggtgattagaatttgggcagagaggctggttataggaaaaataaggaggaagaaatggccttggtttacactgggctaatgaaaccatttgttaaataatgatcaaataaggaaatagtttgtattaaataagtcgaatcgtgctagattatagaggtattatagaggtcttgaaaaccaggggaagaaaattggattgggcttttccttaagcatttgtccttctgattttcaagtgagaataattaatccagtcctcatacaaaaattaatgccaacttatatattattactttttgcatgattatgcgttagaattaattaaatgttacaattttttgtataataaattaggctttttttccttcttttttaggtcaactttcattctatgatgcaaattctaaacagttgctatattcctttaagacaaaatttactcagccagtactacctggtttcatggttagtatgttttatatcttatatatacctaacatattttacttggttggcaactttaaggagaatattctatactgtatatttggagaaggagaatattttgttttttcttcatattctcctccatttccccaattcaccctctcccaaatctgtgattgtttttatatatttttggtatattttattgaagtttatgttaatacatgaagtacacaaatcatgtagtttgatgagtttttataggactgcactcatgtgtaactagcacttagaacattacgagaacctcagaagccccctctagtgcccatttccagtccctaatggcccttctccagtgttagcactgtattgacttttaataccctaaatttacttccttttcagttttatataaacagaatcatacagtatctttttgactcaacattatgcttgtgagattaatccatattctatgtggttatagttcattcattctcatagctgtatagttttccattctgtgactatatcaattgatttataaattttaatttagttggatatgtgggtggtttccatttgggggctatacaaatagaactgctatgaatacttttgttcatatcttttgataaatgtatgtgtatatttccattgagtatatacctatgattggggttgctagatcatatcgtatatgtataatcaactgtaaaattgccggttttctgaaatggttggttatgctaatttacaactagcagtatgtaagaatttgagttccttcaaatccttgtcaacacttagtattatcttttaaaaaattttttgtccttctagtggatgatatattacattttggttttaatttgcatttccttgattactagtgctgttgagcacctttttatatatttgttgactatttgggtatatgcttttgtgaactggctattcagatcttttgcttgtatttctattaggttgtcttcgtgtttcttatgggttaatttgtaggctcttcttcactctggctttcctttttccttattggtattgtttgataaacaaaagttaattttgttcagtttatcaattttttcatttacagttagcactttttgtgttctgtttaagaaatcagtatgcacccccaaggtcatgaaaatattcttctaaaagctttaccttgtacatttagatatagactgcatttacaatgcaagtacaatgtagaattgatgtgtttggtatgaagtaaggatctagatacgttctttaattccccatggatatccagttattccaggaccatttattgacaagatcatagtgcagtgtcatctttgtacaaaatattagatgactgtctttgtgtgctatgctgaatatatgtatgcacaccacatagcaattacatcctgtgtaattgcaggtctactcaatttcaggctgaaaagaaaaatttgtttctctgcacaaaataaaacatggttttgaatttatttaagcaaatgttattgctttttccaactcataaccttctgcatcttttcataggttaggttcccgtggggagttgtgggatccagttaaagttaccattactttggctagagcttttcttaaatttggaggctacctctataagtcaagatggtatatttcaaatggaatattttgcatgtatattcttctgtcatcacccctaactgtaacttcccaactataaggagaaagttttcagagtaagagtgggttgaaaatacagtgcttttaaatctcattatccatagtaattatttattccagatactttaatctcttaagtttaaaacaatgctaataaccaggacacctatttttacattaaaagtaagtgattagtgactaaagttattgctcatggaaacataaagatactggaagggagggttgtttctttttcctttttttttttttttaactttgtacaaacctctgccatattacgcatttttggctatttttccaaactggtccatcaaggatgagttgtttaccatgtggaatgcagaaaaattttttccaagacttaggtgtgcttttataaatagtagatttacttttaatttgaatctatctcatgtatgtatgtactgagtttattgtttttcattccaaataatactctaattatattagtatatgtcataagatactgcaagaaattattttaagcttgttaaaattttttttccttcattgaaggcttgcttttattaagtacgttaatgcctattaaatgttttgtgtacaagattaatttttaagtcagttttattgaatttatagtatggtgcagttctgtggtttttagcaaatgcctgcagttgtataaccaccaccataatcaagatatagaacatttccatcaccctagaaaattcctttgtgttcttttatagtggaccgttccacacaaccagccctagctatcagtaaccagttcgtaggccctatagttgtaccttttccaaaacatcgtataaatagaattgtatggtatgtagcctttcgattccgtaccatgctgcatttgaaattcatccatgttgttgtggtgtcagtattctcctttttttcattgctgagtagtgtttcatatatgtatgtatcacagtttattcattcattcaccagttgaaagacacttgggtttttcccagtttggggcagttatgaataaaatcactataagcatttacatatgggattttcccttgggtaaatacctaagagcagtaatagagtagctgtatcacattgaaagtgtatgtttaacttcatggggaactaccaaaatgttttccaaagtggctgtaccattttttgccttcctatcagtgatatgagagttggtcatatccttgccattatttgatattaccagattttttgttgttgttaagccattttaataggtgtgtagtggtatgtcattgtgtttttatttgtagtttcctaatgacaaatgatgtttcatgtccttatttgccattcatataatttatttcaagtatctgttaaaattatttgcttactttttaggacttaattgttttcttatttttttattttactttatttttaagacagggtctcgctctgtcacccaggctagagtacagtggtgcgatcacagctcactgcagtcacaactgcctgggctcaagtgatcctcccaccttagcctcccgagtagctgggattacaggtgcccaccaccatacccggctatttaaaaaatgtttcttgtacagatggagttttgctatattgcccaggctggtctcaaagtcctgggctcaaatgatccaccagccttggccccccaaaatcctggaattacaggcatgagccactgcctggttttcctgtttttaagagttctttataagtttggatgtgaatcctttgtcagatatatgctttgcaaatattttctcctggttatggtttgcattttcattttctgaacatttcagagagaagtttttcattttgttatgaagtccaatttagtaatttttttccctattatgggtaatgctttgcttaactcaaggtcacaaaggttttatgttttcttcttgatttccctttgcatcttcatgttagatattttgagtaaatatttttctaaatcatttaaataatttccaaaaaataatatagtagttttataatcagaaagttgcttttgtattttgggagttatcattactgagcctgttagttttgaaaatttataatgttaattatataattacaaatttcacagttcagtagattctttggtataataatctagttacttagtagatattgaacacttaagggtataattgaaggtgatgatacttaaacaacttctagaatttcccttgctttaagcttgtgtctactattaatatatacggtagttgatgatagtgtcaatgatctgtattttcatattttaattcttttgactgtgtcccaaatcttatgtctcactttattgaattatagctgctctgttcccaagcagttttaattttattttattttttgtttttatttttattatactttaagttctagggtacatgtgcacaacgtgcaggtttgttatatatgtatacatgtgccatgttggtgtgctgcacccattaactcgtcatttaccttaggtatatctcctaatgctatccctctcccctcccccaaccccacaacaggccccggtgtgtgatgttccccttcctgtgtccatgtgttttcattgttcagttcccacctatgagtgagaacatgtggtgtttggtttttgtccctgcgatagtttgctgagaatgatggtttccagcttcatccatgtccctacaaaggacatgaactcatccttttttatggctgcatagtattccctggtgtatatgtgccacattttcttaatccagtctatcattgatggacatttgggttggttccaagtctttgctattgtgaatagtgccgcaataaacatacatgtgcatgtgtctttatagcagcatgacttataatcctttgggtatacacccagtaatgggatggctgggtcaaatggtatttctagttctagatccctgaggaatcgccacactgtcttccacaatggttgaaccagtttactctcccaccaacagtgtaaaagtgttcctgtttctccacatcctctccagcacctgttgtttcctgactttttaatgatcgccattctaactggtgtgagatggtatctcattgtagttttgatttacatttctctgatggccagtgatgatgagcattttttcatgtgtctgttggctgcataaatgtcttttgagaagtgtctgtccatatcctttgcccactttttgatggggttgtttttttcttgtaaatttgtttgagttctttgtagattctggatattagccctttgtcagatgagtagattgcaaaatttttctcccattctgtaggttgcctgttcactctgatggtagtttcttttgctatgcagaagctcttcagtttaattagctcccatttgtcaattttgtcttttgttgccattgcttttggtgtttcagacatgaagtccttgcccatgcctatgtcctgaatggtattgccttggttttcttctagggtttttatggttttaggtctaacatttaagtctttaatccatcttgaattaatttttgtataaggtgtaaggaagggatccagtttcagctttctacatatggctagccagttttcccagcaccatttgttaaatagggaatcctttccccatttcttgtttttgtcaggtttgtcaaagatcagatggttgttgacgtgtggtattatttctgagggctctgttctgttccattggtctatatctctgttttggtaccagtaccatgctgttttggttcctgtagccttgtagtatagtttgaagtcaggtagcgtgatgcctccagctttgttctttttccttaggattgtcttggcaatgtgggctcttttttggttccatattaactttaaagtagttttttcccattctgtgaagaaagtcagtggtagcttgatggggatggcattaaatctataaattaccttgggcagtatgaccattttcacgatattgattcttcctatccatgagcatggaatgttcttccatttgtttgtgtcctcttttatttcattgagcagtggtttgtagttctccttgaagaggtctttcacatcccgtgtaagttggattcctaggtattttattctctttgaagcaattgtgaatgggagttcactcatgatttggctctctgtttgttattggtgtataggaatgcttgtgatttttgcacattgattttgtatcctgagactttgctgaagttgcttatcagcttaaggagattttgggctgagacaatggggttttctagatatacaatcatgtcatctgcaaacagggacaatttgacttcctcttttcctaactgaataccctttatttctttctcctgcctgattgctctggccagaacttccaacactatgttgaataggagtggtgagagagggcatccctgtcttgtgccagttttcaaagtgaatgcttccagtttttgcccattcagtatgatattggctgtgggtttgtcataaatagctcttattattttgagatatgtaccgtcaatacctaatttattgagagtttttagcatgaagggctgtcgaattttggtaaaggccttttctgcatctattgagataatcatgtggtttttgtctttggttctgtttatatgctggattacgtttattggtttgcgtatgttgaaccagcctaagcaaagcagttttatctttcacaaagtcattcacatttatgataagtaatagaacatgggaagtacatctggatattgggatttgcatttttgtcaggagtccttcttaaataattatataagagttcttatagttaacacggtaaggaagaaaacagtggattttactgttaactgaggggtgttagatttttatagtctcaggccatatctcattatcaaaaccaaaagcataagtgggaagtaagttggtgctttgtatgcttcccttggttgtgaaaattagcatcagtaatgataggtaataccttttgcctagattaagccaatgaagtttctcaatttctgcacccctgagttccttctcttgggtgcagcttcagttggttctgctaccaccaagacctcctctggcctctgtggttctaaaataattctgatttagtctttccatttcccctcagctgaaatatgacagttaatgtgtttgagaatgattgatgttcatatgtgtggcattttgcctttgaaatggaaatttaaaaatcactgaaattctagtttgatttgcaatctgacaggtttttttgtcttttcttaggtatggtgtggtggactttctttgagtactgggatgcaggttccaagtgctgtgagaacacttcagaaaagtgaaaatggaatgactggttcagctagcagcctgaacaatgttgttactcaatagtgtctactcagaatacgtttaccctccgtcttgattaggtggccttttctgtgcagttactaatcacaggaatttggtagtagtgaaaatcaggtttgctgtgttctgctttgaggcctggaatcttttatcattaaacacctagtacgaagcatttgcaggaacctactgtgcagtatcatagaagcaagcagataccaagcaaaaaactgatgattgaagagtaaatgggggaaaaggcagtgtttaattaacataaaaactcatttttgtatttcttggattactttgactattctaatgtttaattacatatggtaaccctaaggcctggggagaaaagcttttaaatcttgccttctttcttctgtactttgtctttttaaaatctcattactatctattatttagttctaacacagaagctttaaaaatacatagtcatccaaggttttctaaaaattgaaatcatatgttgggaatggtaaaaaggttttcaaatggtttatttttcctcttttataaataagttttacaaaattttcctcttttgtttattgactagattgtatataattttcttttttccaaaatattgtgataagaaatttctagacacaacagcttaaaatcacccaaatttcagttctttacctactgcactaacaatggcaaggggggtattctttatatgttgccttgtttaactacagttcttttcattccatcactttaggtgatgggtaagatttttgaaagccttatattttttgattttgttgtctagtttaatcctacctttaatagttgtgtttggtaaaattcccacttgaatgtgacactgataataattatgctgatttttagcatctcttataggaatcaaagtttattaaagttacatagaggattgaaaaatgtatatcactcaatttttatctaagaaggataggttataaagggaggtacctaaatactcaaataatgtatatattctttttcataacatatggaatgctttaagcaattgttttgaaaaaaatctgcgtatctttgacttaattggcacatgactttttcaagcagccattcattcagaggtttgttttctctcagtccttttgctacattcactttcttttcaaagaaatgttaattattacaaaaattgacatagatatctttcccaaacttggggtaaaacccatggttatgtggaacataactgttcttaaaaagtcaattataatttgtaactcacatcctttgagctaaactaaattaaaattacagtatttaataattctttgggcatttttaagaggtctgaatttgtatttttcttcatttttgaaactttacatttgttgactttttttcattctcatttaaaatatattgtgctatgataaccaaccttcttccaaggagtgaccattactgcctacatttgcgttgctttctacatagagacttgtataatagtattaatagtagctcattctctctaaaaatttactgcccactgataggatgttttgtttccttgataaaacaaatgtaaatgaggaattttatttgaattggaatattgtttttctagaggacattcatatctgcactattatctgatgacatgttggtaattttaaagactgcaaggcagtttagagaatgaagtaaaccaatagatactcttttgattctccaaagaaatataattttggtttttgttcctcagagagagtttgaaagaaattttcagatgttctgttccctatagagggcctattccaggatctaaatgaatgggaatttataattcctttcatagactcaaacctgaaagcagaaatttttagtagttgagttgctttaagtgaattttaacaaatatgacacagaaaaggtcagatgctgttgtataaaattttttactagtgtgtcttatataattctttcttctcattaattcagtgcctttttcctctaagcatactcttggtccatgccccatgcagtgtcaactgatgtttaagctacagagcattgttgtagtggtgagggccctctgttgcaggggcatggggaaatgcatatattaatcaggggctggaggagtatacatgattcttgtgttcatgttgtcatttgaaactcttcacataaaattttctaatattcatttggaaaacctctccactggagaggtttcatctctgagaggttttgtaataatagtgtaagttcagtaaatccagtccaaattctcatcacatgtattatttgatactaaattttcaattattacttcaaaataagagtctgaggatttcttcttactggcgttcttaaaggtctctaaaattaaagaacaagatgtggttttttgtttaagacgtttttagtttatttgttgttaagttaaactggagaaagtttgtcatcctcattttcaaactgaaaactaatcaaatatagtgcctatttagtctcaaaataaggtaactattaacttgattatactatataatattctcaattacatttgaatttaaaaatattgagctcttgattacaatttaatacattgtaaaaagtattaaatcctttgaaacatcttttgttgcttatttagtttttgtttctacaggtcaaacatgattgctttctataaaagaaatgcttgagaggttgactataatggatatgtcacaggtataaaacagttgttttctaaaaacatgcatttagtatggcattctcttttagcaactgaattcccaacgagttttattaagctggatatcgaaatgaaggagctgccttaagcactttagaaaaagaatttttttacaattcattttgactctcatggctgaccatgtcattatgtctttaaattttggtaaatatgtagataccaagcattaataactaatgcacacagaaatttaatatacagcaattctttgaatgttccaggtgtacgtaaactaactgaaagtattaaggacatgcctgtctatacatgggtttcattgatggtatctgtatcatcttgacaaatcgtgaactgctgctgtatggctagactttgcctatttactctgttatgcaaacagtaatttttccctatgttatgaagagagacatattggcttgctttaatttacttatttatgaaattaaagcatgaataatatgtataatttgaattttttgtgactgatccttggcagtataaatgataaaagtaaatgtaatggaatcttttaattaggctaagatatgctatttcataacttatgtagaatgatttttatctatatactttgtccataaaattataattgtttatgtaattttattgtttcttatggaaacaattggaaaagtatatggaaaatgattatttcaaagaatatttatttaaagagggaagtgtagacttcttactgtaaaatatgtgattccaggcttaagaaattgattatattttaaaataattatttttttaaaaacgtaatttgtttttaaaagatgagtctccattcattggctaatccatacagcaaatatttgagtgtttgtgatatggcagtaaaaatgtgattactttgtatgtacattaaccaaaaccagtgaagtttgatggactgtgcatagagttttgcagcttttgagtagtgtgacagagtttgcctcttaaaattgttttgctaataagtcagaagtttaaaatgtgttatagtttgctaaaaaaaaatcaaattaactgcatataaaatggttcacttttatatagtcacatgtaatgggcctgaaaaagtttcttctttgattatgtagttactctagatacattcttttagggaagtgtatggtcaacatatatttactcagtatacagataaccacaaagttgttatttttaaccaaaatatacatttcataatgttggcactggagtattataagagatcatgaatgtttccttaattatcatggcaagattacctcacgttcagtatagtttagttttgtgtgtatcttacagtatgcatgttctgaaattatttgtgatcctgatatgtcacatataatagctttgttacctggagtatttgattaacctaaacagtttaagcattttgaattagttggagtttaaatggattacatttggtgtatattgtcttcattgaaaagatattgttggatatgccacatcagagttagcattgacttataaataaataccagaatttaccagagtacacttttctcttcagatgactcaattattaaataaaagaatatttcttatttctgggtcaatataaggtactgacttctgatgcataatcacttaagctatgtgagtttaaactggtatcttttcttagtggtacccattcaatgtaagctggtccatgggaatggacatgaagaggatttcacagtatgtagagcagaaggcacgtgaatgtgtttgctttggcttggagcttattaagttttgactacggttaaaataagtcaaatagtaagtggtaaaacacatttttgttagtattggaactttctggagaacataagggctatgagaatgcatatatatattttttaacatttcctatatatctaaggtaccaaagcactgagtctaatttacctattaagggagactctttaaaatcaactttataactaattcatactataagacagataatagctaaagttttggaataatttatattaaaagccgcaagtcttaaaaatccctggatatgacataaaaaggattttggcttcttttttgaagtatttaaaattaatcaccttagctctaccatatactagatttgtgaccgctacacaaattgtttatcatctttgggtctctattgccttctttataaaataagtgtaagttgttcagcctgcctcacagggctgttgtgaggaaataaaatgaaatggagtatgtgaaattgcttcagcaacagcaaagtgctacgtaaatgtaaagtgttgtttttagctaataatggatttaagtgtttggataattgtagatgcatttactttgataaagcgtgtgcttaaagtggtatcaccagtgatttctaacatgattttaaaaaaataaaaccccaattaaaatgttctttaatattcatttaatttgtgcatgacttgtggcctttttgtattttctcaagcctattactctagagctgtaaaagctcttgcacagcattgttgtgtcagtgtagaatagtggcataaataaatgaattaagctacatttccatgcaggcatttgcactttgaagttagggctgcccagtgccacatgcaaagagtgtatttggtctaaacagttctttccaaacaaccaaatggctgggcagcttgttgtcacggataaatgatataaaatgtaaccactgaacatttgacaactttgttgcattatcatttttaaaaaaagatgaagcatttcaaaatcttgttaacctggttatctcttggtatctctcctgacatatttgttttgctttaaattggattaaatggtttacaggttatctgaatctacagatttagtatgtctattatctggacatgattttgctatgcagttgtgataataaaaattctaattcctcaggtttggccttttaagttatggctgaagacctttaatgaactacttatgatgcattcagtgccatacaatagtgttttaagaagcacatggcctcattttccttagaaacaagacaaagcctttttaaaatgtttttttttcactttaaaatagggtattcaaagtggagtaacgtgtattttgaaatgattttgtgttctatatagaatgtcccagttaagattttacagaagcacctggaatatctcattaaaaatttaaaaactcttttcctgctctcttttgcttcattgtttgattttattaacttttatttaagtataaatacaatatgctgttggggatgagaatataaaaaaagtcatagttcctttgcctaaaaagcttaacattttagagcactactgttcaacagaattttatgcaattatgaaaagttatttgtgcagtccaatacagtagtgactggccataggcagctactgagcactttatatgtggctacatagagttgcatattgctaatagccactgttttgaacagtgtacctacagatggaaaatgaaacatgctatgttagtaactataatattacttatgaatttggtttctttggatcttgttacatgttgggttacattttggtagatggtaactaagagtcagaatcagaacctaaacatttttaaaattcttgctctaacttgaaaacagtttaaaagaaaaaaaatcagtgagactggagcacctgtaactaagaagttatgtaagaagaatgaaaggagactggatagtcttgagtcacaggaagaagaatggacaaagattgataaaccactatagaagatggagagtgaatgggtgcagcatttctggagaacaattttagcaatattaagatttttaaatgcacatgctccttaatttcctttataagtatttctcttacatatatactcacaaaaaagccaatgttccttgcagcattaccatagctaatagtagcaacctaattattaattgaagacctacaaatttggatggacttggaggtaaattccttttccttttttggtagcaaggcacagaactggttcaaaaggcccaagttgcctcaacaaaagaatgtgataacagaattttgaaggctccccttttctaacttgctgcaccagcaaactaccatataagtagtggtctagatattatatattctgcacattcccctccccaataaatgttatatagaccattatgacaattggcttaattagagccttttccttggtataccagttcatttgtgcctggctgggagttctgtggcataagagctcaggatattatgtgcactctacttttctactaaaccccattttacacttacactgcatggtgtatttgtatttatttatttttgcacaaggtcggcacaagagcagatggttagattttggtatttccatgtgatcctacacagctgttaaaggatatgctgttaatggaagtgtattcatgatattaaacaaaaaagtcatccagcaatatatacagtacgatacaacgggtgtgtgcatgcatgtatacttgggtaagaggggaccctgacctgatcaccacacagtcttgctgtgcttctcttcatgggatgaaaaattgaggagccaagggattatgcctacttggaatgcatgtttcattacccacttatatactatattattgaaacagtctttcgttgtctgagataacacctggagttcttgtccacttatatactacattattgaaacagtctttcgttgtctgagataacacctggagttcttgtcccacctccaagacgattatggagcacggacacaaaggtgaggttagagtgaaagtttaataaggtgaaagaagaaagctctctgccagcagagagggggtcccgaacgggagtgcccatcatgaggctggggtccaggtttttatggacggaaggggaaggaatgtgcttagtctgggggctgtcttggcgaatgcgtgactcggcttggcccgggaccagtcaggaggtgaaatgattcatagatgctgcttagcttggcccaggacctatcagaagctgaagtgaagtgtggccgaggaccaatcgggctgaggtgatgatacacagcagctggacttacagtcctaacaaaggaaagtagagcgcccatagaaacttacgagagcccactgtgcccatgcctacaaaaggggaataaacttttcctgggaacctgctgacaatacaaaggaccaaggcatttctatgccaggccttgttcccttatctgagtgagctggaggtttgtgcaagtttttatccaaatgggccgtaggtttttccatctgtgcagtcatgggcatgtctccaggcacaacaccctgtgctagttcccttattggtgcctgcagcttttttcccaggctgctttttatattatctggggataaggcactgactcatgagccaggggctctccaggacccttctcttgttacctacctaaggtaagctaactaaccggatccccacactcttgctgtgcctctcttcatgggatgaaaaattgaggagccaagggactatgcctacttggaatccatgttcctttacccacagaattctatactatgttatcagccagaaccccaggattccttgcctcatcagcctgaagcttgcttccaggatatgtgcaggccttttgtccaaatccatcctgaaaaaagactactacagatgtatatacccctatggctggcagtttgtgggaagtacagatgaagcttggatgtgcagactgagttgtccacatgcatgcatgataggcccctgtggcaggcttaagctagaagtaaaaagagacccaggggatcagggaagggcaggccaacctagtatcactttctagtacacttctgaagaatctgcgaatcgcatatttgaacctagatttctgttccttgagaatacatgttaaagtagaagagtataacattttatttgttggttaacgctcagctatttagacactgaaaatatgtcagggttggctttcatttgtattcttggcccagaccctacaaatgttaggagtcggccaggatccttacatgtgtgcacagctgagtggtttatagaacatgaatatttacttgtaagagaggctgtttttatgcatccttgtacccactctttcagctgtatttgctatccagattaaagcatactgacttgacgtttgccatgagctgagggctcacatttgacctttcagtatgcttgataagtaacactgccaccagtttagttgtatatttaccttcagttatgtttgttcccaaacctgcttatgtaggtggtagtcactgttgtagtcatgtaagtatgtaaaccaattatataaatatataaaccaaaataaatatgaaatgagtatgaaaaggtacttataagaaaagtacgagaaccattagagatgaagagtttaaaaagttgcaaagttagttgtggccaaagtaattgtgagtgataggggaagatttttaaaaataaattccaggactccaaatttatattccttcacttgtatctttaagttcctggtccattttacagaaacagaaactacaaatgatggatgatgcattatgtctatggttttgtaagaaaaacagtgagatactctaatcagctggtccatgcttaaaatgaacttagttcaaaacagaagattggccattgtaaccctctactgaaactgcctttttgagaaggtttattcagaactagatttgttatacacttggaaagtatttatttctaagaacctgataatttttcccttttcctgttacttttaattataatttccaaatatacagaaaagtagaaagccagtgctttgtgctcatcacctaatcaattgttaacattttgccatgtttgtgctatctattttgttttaaaatgtcacctgtaagtatgctatatgcatccatgatggcttttaaaaacagccacattctgttaacattcttagcaaaattaacagtaattctgtactattatctaatggatcagtccatactaaaatttcagttgtctcagaagtatctttttacagttatcttgttcaaatcaagatctagacagggtccacacattgtactccgttacatctcttaaatatttgattttacaatagttccctctgcttttaaatgccatttatgaaaaaaactgaggaatttgtctggtagaatgtcccgttttctgaatttagttgcttctctatatcctgtattagatctagagtttgagtaaatgcaggttcaatttttaggcaagaatccttcacaggtgtggctgtgtactttctatcacatcaggaagtacataatatatgcttgtcccaaatttagtgagattaagatcagtgggtttaggtgatgccagtctattataaagttccccatcaacctttcaccttaattttatcatctattgatgttgccctttcgattattttattaggagttacaaaatcgtgattgttttatcatcctccatttattagctggaactcttataagtactttggttacactaaaattcaattcatacaagaaagacaggataaatgcttgatgttttcccttatcaagttttagaatatttaatcttcaacttggcaatcttcaatcacgactgaattttattttttaaggagtcattataaactcaagaatttttatatttgatgtgtttcaatcaatagcaagtatgtgatgctcaagttttcccatgtcccatcacgttagcacctgtgttaatgatgccattaagctttgataacttacttcctcttggtgtaaccttccacttttttttattaacctactgagtacctacccgttctgagtgcattggatgagaggacttcaacagtaagcttgtatgtgcataggaaatttctggaaggaaaaacaaaaagttggtaaatgtcataacctgtaggaagtgaggaagattttttcttccttttctttctgtactgatagaattaaaaacaaagcttagaaaacaaatatatgatgggagtattttccgttttgtagaaataaattataattacagtaactggtttagtgaattatggttttcaaaaatttataagaagattaatatctgagccttaacaaccaccttttggattacaccgttaaaagaaccaaagtgagaggatcgcttgaggccaagagttcgagaccagcctgggcaagatggtgaggacgccctcccccccacccccgccacaccccgccctgctagcccccaacgtctctacaaaaaaagaaaagaaaaaagttaatcaggtacaaaattgtatccagccttaaactggagggcaacaggtcgctaaatcttgaatgtcataaaggcacctcaacttcatgaggaatagtgaacgcagctgctattttccactctatcccctagctctactaattgtatccaaaccaaacttcagggagttatgctgaatccctctagcaaagcacacgcactaaaaaaaccactcgtttatcagaagttcacatttaacgggcttggaaaacggctcagctgctgcctccagttcatcttccgctgtcgaaagcgtttcagaacttaaactctcagattgcctcagtgcgctgctgtagttgtcaattaggcaagagataaaaaagggctttggctaagtggctagattataaaagcgaggaatcgccagggctcagtgaacttctggcggtgaggatgcgacaagagtcacaggaaagccgaggctggggctggaccgtgggaacgtcccagcaggaaccaagccagcctccgccgctcagcacttgacggcggcttttgcggcggttgctgtgagtgccgtaaagcggagcggctgcagcctgctgttgagtgaggtaaggtacgggaggctcaggtcggtacccggggatgggtgggcgccttcagacaggtaccgctggcgactcgggtgcccttaccgggcatcctccagcattctgggcacctgcctaccccttggtgaggaggccggccacaggctgagcgcgctccgggctgggtactcctcagtcagtccacgagcatcgcgtggtagacttccacttggccagtccttcccgcacttctgggcgtgtcatcaggtgaaatcttaatcctgggacagatgaaaggttggaggacgatcgagactcttgtagtagccgggttagggtagtgacccctgacctcaggttatccgcccgcgttggcctctcaaagtgctgagattacagccgtgagccaccgcgcccggcctgaaatttacaatttctcatttaacatgaggtaagccacatttctcttggcttcagttttgtcagatgtggaaaaaaaaaaaaaaggacctagatgatatatcagattctttatgcttttgaagatagcacgtttccagtcagtaaaaatcaagctgtgaacaaatgacaaagtgaatgatagagcagtatattagaaattgggcagatggaagcccagtagaaaaggctgtgtttgagctagactctgaggataaatagggtttgaacgattggaaaccatctctgttgggccatggacaaagatatcaaatgcaggaataagcatttatattttagcgattctatttgtggacataagtttagtgagggtagaggatttgggaaggctggcattgaacggtgaaagaactcttagtggaaaggaagtgcagggtgttctgacaaggaagaagaaaggaaccggggaaatgccgaaagaacaatacgcaggacttgatttcttggatctgggtgatgatatttttaacctgcgtttctaaaaagtaagtttaagtgctgttggcaaaaatgggaattctgttgaattccagcatgcaatagtgtactgggaataaagtgatttagatcgtagagtgctgaggttgccaataactagcctcttggctgtcatttaattcttctagagcctattctccataaggtgatgttgggccagctgatctctcttctctaaagcctgtaaaactagagactgtgaggatggagagctagttactttcttctggactgggagaggacgatagttgacagagaataaaattgttaattttggggctggacgcggtggctcacgcctgtaatcccagcactttgggaggctgaggcgggtggatcacctgaggccaaggagttcgaaaccagcctggccaacatggtgaaaccctatctctactaaaaatacaacaaattagccgggtgtggtggcgggcgcctgtaatcccagctactcctgaggctgaggcaggagaatcgcttgaacttgggaggcagaggttgcagtgagccaagatcaggccactgcactccggcctgggcaacaagagcgaaactctgtctcaaaaaaaaaaaaaagttaattttgaacatgttaaatttgaggtgaggtgcaggaaatagagttgaaaatataggcagatagagtgcatggactgtaatttaaatagtgttttctctcacaggtggtagttaaaatcttgagaatggatttgctttcagggagagattgtagagagagtaactataggccatacccacagagaggaggttggagaaattattgaaggaggcatgtggatctcagagctaagagcaaggaaggagttctttttaaaaaagttacatatagttgtagattctcaggggcccagtgttgttattaagctaatttaacagcatttacagcaaataataagcacctacttctgggaattctggcagaaaataaataattcaaatagatataatctccactgcctaattgtctacccagaagtggtatcatttacatatttatttattcaacaaatatttatatgtttcaagcactgctggttctagggatataacgacgagcaaggtagacattgttcttatcctccctgcatgtaaagcccttagcatctacatcagtgcttttcaaattttaatgtacatatgaatcatctgaggattttattaaaatgtagattatgaatcagtaggtgggggctgaaaattctgtattactaacaagctccaatgtgatactgatgttcttaggaccatacttttaagtgacaagaatctagatcctgtttagcaaatatggccgttattaagccactaccactacccatcatctgtttctcctaggataaaataattttacttcttatgaaaataatatatgcttatacaaatattggaacaatatagaaaagtgtaaagaaccatgtaaaaatcactcctaattctccctacccagagataaccattattaatatttttgggaacattcatccagattttacatatgtacatacattcacaatttaagtgttgcactaagtacatgtcacactctaagccctgtgtttgattctatttgctgtatgattttattaagataaatacccaagtgtccagaaccaagcaattaagtacttgcattcttgagggagccacttaaaaataatttgggggccaggcacggtggctcacgtctgtaatctcagcactttgggaggccaaggtggatggatcacgaggtcaagagatcaagaccatcctggccagcctgatgaaaccctgtctctactgaaaatacaaaaattagctaggcttggtggcacatgcctgtagtcccagctactcgggaggctgaggtaggagaatcacttgaacctgggagcggaggttgcagtgagctgagattgtgccactgcactccagcctggcaacagagcaagaatccgtctcaaaaaacaaaaaaaaaaacaaaacaaaaaacaaactttgggagccggacagtgtctcatgcctataatcattccaggtgcccaagaggctgaggtgggaggattgcttgtgcctagcagtttgaggcagcagtgagctatgattgtgacactgcactccagcctgggtgacagagcaagactccatttcttaaaaaaataaaaacttgtgttacttcaaaaatggggagacattaacataattacatgtgggctctagtaaatgaatatttgtcatttcatttaggatgagaggagaatttttaaagttttaaaaaaaacttagtttttttcttactacaaaatcaattgatgttcacgtaagataaataaggaaaaaaaataaaagcacctacactcctcccaacccaaagacaatccttgctgtcttcaccttccttcctgctaacctgtcttatctatatctttcatttcagccactatctttccaaaaccctcttacaccatagtcattcagaaaggagtaactatgtatttatgatttttctggagcatctactggagaaactaaatttcattagctttttatcttcaagtaacagcatgtgtaggtagaagttatattgcaaaggattaagtgcatgaatggtaagcaggtaaagaaacttcttaaccctttgcagtctaatgtttacttccaagctgctgacagttgtgaaaagttagcagtcaaaggaaaagaaatggacaataagaaagaccaacagtatttagggaagatttgatagtagctgttgctactgggatatttttggcttttgagaacagctgaaaaatgtcgatttttttttttttttggtctgacctctgaattcattttcagacgcattttctctttatgcctgccaatctgctacatcatctctctaactataccttttcctaattacactactctctttcctctgtagttcagcctcctgttttattttgttcagagcatatttgaatgtcagttctgttttaatgaattgcctgaaggattcttcctgtgcgctgcacaaacgaaaccagttcactgagaccgtgctactgcagtaaagaaacagcttacttaacaatgatgctggctgtgcaaaggagttattactcaaatcagtctcgccaaagacttggtggttagtttttcaaggatagtttttagtttggtggcaggggactagggaatgagggctgctggttggctggggatgtgatgataagggtgtgaaaaatggtccttgtgtgctgagtccacctctgggtggggagccacgtgactggttgggtcatgagtcactagttcacctctaggtagtgtcagttggtccagaatgcaaaggtctgaaaaatatctcaaaagaccaatcttaggttctgtagccagggaaaatataaatcctgtgtcctctggaaaaaagactggttatcatttaactacatgttaccagaattcaggtccctctcataatcctaatcttgtagtctttcattacctttataaaggcagtttagttttggaaaaggttactatcatccttgctttaggttaaactgtaaactaaattcctttcaaagttagcttggcctgcacccagaaatgaccaaggacagattggaggtcagaaacaagatggaatcaactatgagatttctcttagctgtcataattttgcaaaggcagtttcactctctgattcatactatctatgcctcactcttactccccaatatccccaaataagtcggggatcccacagcataaggatatggctaggctctcacatatcatcttatgaacctaagttaggtgtcagggaaggtttttgattccacttccccccactcctgccttctggatcatctctcttgatatatcattcattcattcattcattcaaacagacccctacctaggtgattctcaaaagagtggggtctggggctggaggaggtgtcagggtaaaccagttaccaaaagtctttcatactaataccttcaaaggacaaatgcaaatgtaaaaaggaagctgaaagaatatgcagtggggttccaagatggccgaataggaacagctccagtctacagctcccagcgtgagcgacgcagaagacgggtgatttctgcatttctaactgagatactgagttcatctcactggggattatcggacagtgggtgcaggacagtgggtgcagcgcaccgagcgtgagccgaagcagggcaaggcatcacctcacccgggaagtgcaaggggtcagggaattccctttcctagccaagggaaggggggacaaatggcacctggaaaatcgggtcactcccaccctaatactgtgcttttccgacagtcttagcaaacagcacaccaggagattatatcccacgcctggctcggagggtcctatgcccacggagcctcactcatttgtagcacagcagtctgagattgaactgcaacgtggcagcgaggctggggggggggcacccgccattgctgaggcttgagtagataaacagaggggccgggaagctcgaactgggtggagcccaccacagctcaaggaggcctgcctgcctctgtagacttcacctctgggggcagggcatagccaaacaaaaggcagcagaaacctctgcagacttaaatgttcctgtctgacagcttggaagagagtagtggttctcccagcatggagcttgagatctgagaacggacagactgcctcctcaagtgggtccctgaccctcaagtagcctaactgggaggcaccccacagtaggggcagactgacacctcacacagccgggtacccctctgagacgaaacttccagaggaacgatcaggcagcaacatttgctgttcagcaatattcgctgttctgcagcctctgctgatacccaggcaaacaggatctggagtggacctccagcaaactccaacagacctgcatctgagggtcctgactgttagaaggaaaactaacaaacagaaaggacatccacatcaaaacccatttgtacatcaccatcatcaaagaccaaaagtagataaaaccacaaagatggggaaaaaacagagcagaaaaactgaaaattctaaaaatcagagcacctctcctcctccaaaggaacgcagctcctcaccagcaatggaacaaagctggatggagaatgactttgacaagttgagagaagaaggcttcagacgatcaaacttctccgagctaaaggaggaagttcagacccaacacaaagaagttaaaaaccttgaaaaaagattagacgaatggctaactagaataaccaatgcagagaagtccttaaaggacctgatggagctgaaaaccatagcacgagaactacatgaagaatgcacaagcttcagtagccgatttgatcaactggaagaaagggtatcagtgatggaagatcaaatgaatgaaatgaagccagaagagaagtttagagaaaaaagaataaaccgaaatgaacaaagcctccaagaaatatgggactatgtgaaaagaccaaatctgcgtccgattggtgtacctgaaagtgacagggagaatggaaccaagttggaaagtactttgcaggatattatccaggagaacttccccaacctagcaaggcaggccaacattcaaattcaggaagtacagagaatgccacaaagatactcctcgagaagagcaactccaaaacacgtaattgtcagattcaccaaagttgaaatgaaggaaaaaatgttaagggcagccagagagaaaggtcgggttacccacaaagggaagcccatcagactaacagctgatctctcggcaggaactctacaagccagaagagagtgtgggccaatattcaacattcttaaagaaaagaatcttcaacccagaatttcatatccagccaaactaagcttcataagtgaaggagaaataaaatcctttacagacaagcaaatgctgagagattttgtcaccaccaggcctgccctaaaagagctcctgaagggagcactaaacatggaaaggaacagccgataccagcctctgcaaaaacatgccagattctaaagaccatggatgctaggcagaaactgcatcaactaacgaggaaaatcagcagctaacatcataatgacaggatcaaattcacacataacaatgttaaccttaaatgtaaatgggctaaatgccccaagtaaaagacacagactggcaaattggataaagagtcaagacccaccagtgtgctgtattcaggaaacccatctcacatgcaaagacacacataggctcaaaataaagggatggaggaagatctaccaagcaaatggaaaacaaaaaaaggtaggggttgcaatcctagtctctgataaaacagactttaaaccaacaaagatcaaaagagacaaagaaggccattacataatggtaaagggatcaattcaacaagaagagctaactgtcttaaatatatatgcacccaatacaggagcacccagattcataaagcaagtcctgtgtgacctacaaagagacttagactcccatacaataataatgggagactttaacaccctactgtcaacattagacagatcaacgagacagaaagttaacaaggatatccaggaattgaactcaactctgcagcaagtggacctaatagacatctatagaactctccaccccaaatcaacagaatatacattcttctcagcaccacaccacacttactccaaagttgaccacatatatggaagtaaagcactcctcagcaaatgcaaaagaacagaaattataacaaactgtctctcagaccacagtgcaatcaaactagaactcaggattaagaaactcactcaaaaccgctcaaatacatggaaactgaacaacctgctcctgaatgactactgggtacataacaaaatgaaggcagaaataaagatgtgctttgaaaccaaggagaacaaagacacaacataccagaatctctgggacatgtttaaagcaatgtgtagagggaaatttatagcactaaatgcccacaagagaaagcaggaaagatctaaaattgacaccctaacatcacaattaaaagaactagagaagcaagagcaaacacattcaaaagctaacagaaggcaagaaataactaagatcagagcagaactgcaggagatacagacacaaaaaacccttcaaaaaatcaatgaattcaggagctggttttttgaaaaggtcaacaaaattgatagaccactagcaagactaataaagaagaaaagagagaagaatgaaatagacgcaataaaaaacgataaaggggatatcaccaccgatcccaccgaaatacaaactaccatcagagaataaacacctctacacaaataaactagaaaatctagaagaaatggataaattccttgacacacacactctcccaagactaaaccaggaagaagttgattctctgaatagaccaataacaggctctgaaattgaggcaataattaatagcttaccaaccaaaaaaagtccaggaccagatggattcacagccgaattctaccagaggtacaaggaggagctggtaccattccttctgaaattattccaatcaacagaaaaagagggaatcctccctaactcattttatgaggccagcatcatcctgataccaaagcctggcagagacataacaaaaaaagagaattttagatcaatatccctgatgaacatcgatgcaaaaatcctcaataaaatactggcaaaccgagtccagaagcacatcaaaaagcttatccaccatgatcaagtgggcttcatccccaggatgcaaggctggttcaacatacataaatcagtaaatgtaatccaacatataaacagaaccaacaacaaaagccacataagattatctcaatagatgcagaaaaggcctttgacaaaattcaacaactcttcatgctaaaaagtctcaataaattaggtattgatgggacgtatctcaaaataataggagctgtttatgacaaacccacagccaatatcatactgaatgggcaaaaactggaagcattccctttgaaaactggcacaagacagggatgccctctctcaccactcctattcagcatggtgttggaggttctggccagggcaatcaggcaggagaaagaaataaaagatatttagttaggaaaagaggaagtcaaattgtccctgtttgcagatgacatgattgtatatctagaaaaccccattgtctcagcccaaaatctccttaagctgataagcaacttcagcaaagtctcaggatacaaaatcaatgtgcaaaaatcacaagcattcttatacaccaaataacagagagccaaatcatgagtgaactcccattcacaattgcttcaaagagaataaaatacctaggaatccaacttacaagggatgtgaaggacctctttaaggagaagtacaaaccactgctcaacgaaataaaagaggacacaaacaaatggaagaacattctatgctcatggataggaagaatcgatatcttgaaaatggccatactgcccaaggtaatttatagattcagtgccatccccatcaagctaccaatgactttcttcacagaattggaaaaaactactttagagttcatatggaagcaaaaaagagcccgccttgccaagtcaatcctaagctaaaagaacaaagctggaggcatcgcgctacctgacttcaaactatactacaaggctacagtaaccaaaacagcatggtactggtaccaaaacagagatatagaacaatggaacagaacggagccctcagaagtaataccacacatctacaactatctgatctttgacaaaactgataaaaacaagaaatggggaaaggattccctatttaacaaatggtgctgggaaaactggctagccatatgtagaaagctgaaactggatcccttccttacaccttatacaaaaattaattcaagatggattaaagacttaaatgttagacctaaaaccataaaaaccctagaagaaaaccaaggcaataccattcaggacataggcatgggcaaggacttcatgtctgaaacaccaaaagcaatggcaacaaaagacaaaattgacaaaagggagctaattaaactgaagagcttctgcatagcaaaagaaactaccatcagagtgaacaggcaacctacagaatgggagaaaatttttgcaatctactcatctgacaaagggctaatacccagaatctacaaagaactcaaacaaatttacaagaaaaaaacaaccccatcaacaagtgggcaaaggatatgaacagacacttctcaaaagaagacatttatgcagccaacagacacatgaaaaaatgctcatcatcactggccatcagagaaatgcaaatcaaaaccatgataagataccatctcacaccagttagaatggcgatcattaaaaagtcaggaaacaacaggtgctggagaggatgtggagaaataggaacactttcacactgttggtgggagagtaaactggttcaaccattgtggaagacagtgtggtgattcctctgggatctagaactagaaataccatttgacccagtgatcccattactgggtatatacccaaaggattataagtcatgctgctataaagacacatgcacatgtatgtttattgtggcactattcacaatagcaaagacctggaaccaacccagatgtccatcagtgatagaccggattaagaaaatgtagcacatatacaccatgaaatattatgcagccataaaaaaggatgagttcatgtcctttgtagggacatggatgaagctggaaaccatcattctcagcaaactatctcaaggacagaaaaccaaacatcgcatgttctcactcataggtgggaactgaacaatgagaacacttggtcacaggaagggggacatcacacaccggggcctgttgtgggatgggagcaagggggaggcgtagcattggtagatatacctaatgtaaatgatgagttaatgggtacagcacaccaacatggcacatgtatacatatgtaacaaacctgcatgttgtgcacatgtaccctagagcttaaaatataataataaaaaaaataagtaaataaaaaagaatatgcagtgctgctcttcactgtagaaagagcctgagaattatcttgaactccaaatcctgtaccttttttcatcacagttgtgtatgggttttatctactactagtttttttccaagccttttcacatcttgacacatagtaaatttgaccaagaaaagatgaaaggaaacataaaagaatgtgttcttggctggagatgacctactcttggggtctagctgccccaaagactgagaggattgttaactctgacacctataacccattcatgatttagttggtaagcagatctgcccatttctttcttcttcattgccagatctcagttcatgcactagttatgccctgcttccacttcatctaagaataattctgtgtcgcaatataccataattatatattaatcttctcatatttgcattagaactttaagattattgggctacttaaacttcgtaactcccctcgttacatcttttttttccctgaaaacatttgtcatttctctcccaaccactgcctcattttaatttactatctctgcaatactttttcttttcttttccattagagatgatatgctgtcttctttaggaaactttacctaagtgtaagtaaggaaatgaatgctatcctccctagtgtttttattatgatagctaaaatgtaacatataaaaagaagtgtatatagaaacaatatttttgttttagttctatgccatatctctctgtaggttattttttatatttttaaacgtttattttttgaaggttggaaccagatatgtgagtttaaggggctttaaactcttttaaaaatcttttttttttatatttcaaattctgttttattgtaaaagttcctgcagaacagaaaagttttatttaaatagttttctgttttcttgagcattgtgcagtgtatttttagtatacttagcatacttactattacttgatgttaattcagccaattttaggctggtggggaagatgattcatgtacactaacagttataatgcaaaatagaaactagtaaaagcctcaaggttagttgcctctccttgtgcttccatagtaacccgtgcttattccttcattgcaactatactgtattgttattgcctctatatttatctctgatagagtccatcataaactagaacagtggttcttaattgatgtgggggtggtaaggaatggggcttgcgcattttggaaaacatcttctcatattctttttcaggtacatcactctctccaccactatcactactgcccttcttcttttgaaaactcctgtactcacctttaagcccttcaaaattagggaagtgtatcttatttgtcattttatctctagtgcttagcatttttttttggcatctgtgcccattaaggtagacagtaactgtttatttgttgcaggaaggtaaaactaggttggaggtggagggagcacttctaacctggaagaatattgaagacttccttgaagaagtgtcatttgagaggagctatgaaaagaaagtaaactggttttatggaagtaaatgagaacattgcagacaagaggtaatgggcaaaaacacagaggcaggaaagtgtaggatgtattccaggaatactcatgcaaaaaccatagactatgtgaagtgtgagaaagcttatagtaaatttgcctgtattcagtcagattgtgaatacccctttataccattatatgtaatttgaactatttgtaggtggtagggaactattgaaaagttttgattgtggtgtaacttgatttatctgtcagcaacttgatacatctgtcagtgtataggtaagattgtggatacagagaaagtggagacagggacatcagttaaaattaggacattaggtacaattagagtttagaatgacagtgaagaaggaaggaattgatgcaagaggtattttaaaggtaaaatcaacatactatggcttctttttttcagtatcacattattcatttttaagtggttactgaatattcctaatgaagcggtagtgctagtgaaaaggaacattttgataggcgaatctttctcttttgtgactgaattgccttggcatttatagaaaataaataatgaagttaattggatatcatcttgataataaaaatgtaattaagtttttgatattatggtttggaggtttattttataagaattagttgtaaactagagaagaaagaacaagatattaatttagattttatgcctgtagtagcttatataggcaggcctattatgtgttctttcccatttattaatttgggcttagaagaagctgagttatggcctactctgagtgccactttagatttcactaggaatcagcatagaatacattaatgcactgtttaatacaagtacaagaacttgagttgaaatcttgaaaatgaagggcagtctccttgttaatcttgtgagctgccctcatcagagtataggttgagcatcccaaatctgaaaattcaaaatctgaaatgctccaaaatctgcaacttttgcgtgctaatatgatgctgaaaggaatgttcattggagcatttcagaattttggattagggatgttcaactggtaagtgtaatccaaatattctggaatcctaagaagtccaaaatacttttggtcccaagcattttggataagggatactaaacctctatttgataattgtatttccatgggttttaactgaatacaaaaactaataccatcatcaatgttgattgatattgttttcacagttttgggagatacaaaataattatgatttattaggttatcgttgcttaatatacattactgatcaggtgaattgttcacatcactattggtattatttctcttaagtagtttcttgagactgtatatatatatatatatattttagtgtttgctttatatagtcatcagctctggcagctcatttggattgttttaaaaccccaaaccaagacttgattttaagatggtaaagacatttgtgccctattctatctgaaattaccatgaaacaacaaggaaactgagagaaagagatgtaattacatctttgctgagactagaagacctgtaactccaaactgaaatatttgagaaatggcagccacatgtaagcaggaagaggttaaaagagaatgctggtagaaagagatctcagatagagctggcagagcaaagagtcctcttctgtttgcagtgggatcaggatgcatagaaaggcaatgggaatttccttggattgtttggcaacatgaactagcaagaaaggaagagtgaatgaggaagtgcacagataccccatctttgcaggaagcactctcttgctgaggcaaagtagaggagagatagtgagtggccctttgctgcctgtctctgacatctggaagaagtaatgtttaaatgcttttcccacttgttctcatacacattctctgcctttctcacatatacacatgtacaaaatactctgtcagaaagagttttcttgtataccagagactaccctctagtctagaatacacccttatttctttcttccatagttaaggcgtaaattatattcccatttagaaaagtaggtgaggactgggtgccgtggctcatgcctgtaatcccagcactttgggaggctgaggcaggtgggttgcttgaggtgaggagttcgtgaccagcctgaccaccacagaaaaaccccgtctaaactaaatatacaaaaattagccgagtgtggtggcaggcacctgtaatcccagttactcgggaggctgagataggagaattgcttgaacccaggaggtgaaggttgcagtgaactgagatcgtgccactgcactccatccagcctgagtgacagagggagactctgtctcaaaaaaaaaaaatgcttaattgcagttctgaaaatagagaattcaatgttataacagaaaaaatatttaagaaaaccttctgcaaagaaaagacatctttaggtcaggctcagtagtagctcacacctgtaattccagcactttgggaggctaaggcaggaggttctcttgaggctgggagtttaagaccagcttgggcaacatagcaagaccctgtctttacaaataaatttttaaaaaattagctgggcatggtggcacatacttttactcatggctactcaggaggctgagataggaagatcacttaagtgtgggagtttcgggttacaatgagctatgattgcaccattatacttcagcctggacgacaaagtgagaccctgtctcaaaaaaaaaaaaatctttattctacagattgaaaggaaacacactgaatgaggaaaaactaacatacggtcatcaacatccttgtataacctagtttttaaaaaaattggatttcaaaggtaaggaatgcattctttgctcatcccaataaaaagattaaactacctatcaggagttggtttgggaaatcagatattgtcaagggaatatttagcactacaggacaatggtacaaagtgtgtaagtcattggggaaagacagtgtaacctcaaagccaaattgacaactatttttgaacaaggcaaaagctcaaggtaagtggtacccctaagttctttttgataaactgcaagaagatgaatatcagtcatacagtagatgaacagagatgatatagcaaatggattggcagggaacattgtaggaataagaccaaaataactatgagatttgtagttatagaatacaatagaactgtaacatgtagaaataattaataaaagtcaagattgaaagaggagagaagacagaatgtagtataaatttgttggtttcttcttattttatagctggagaacaaaagacatataaaccttagatatcaagcataagagaggtgtcagtatatttgaaggattgaaggaataaatgtaagcatttgaagaactaaatgtgtttaaccaaaatcaaacagtggagacaaggtaggaagaagtagaactgtattaaatttcttatcctaaaggaataatcagagatgagacctaagatgaaagaacaaaatgtttattgtggcattctttacagttgaaaaaactgaaaacatacatggagtataaataaaaactgaccacatcctagatcacacacaaacttgaaaagcaacaaagagctgtcttacaggccatgttccttgactaaaaacggtctcagtttctcctttggaagtggttctcagcattgtcagcagcaccagcatcatttgggaacttgtcagaaatgaaaattctgaggtctcataccggatttactgaatcagaaactggaggagaaaagcacctctcaaccttgttggtcagtttttataaatatcctatttatgttttcagttatttacagttataaaaaaaagtgataataaacatttttgttttttcatcattggtctcatatttgattatttctttagcatagacaatgaccagatcaaagaatgcctgtggaaatttaattttttctttgttctattgttggttattacaggtacaaaattaaagaggtttttgtttctttaaaaatatcttttttgttcacagaaaacaaaattatcttcctttccaaatccaaaaagatgaaaacgactgagatactttcaaaagacaaccaagtgagcagcacagactaatgagtagaatcaataagaacgtggttttggcccttttaacgctgacaagttctgcatttctgctgtttcagttgtactactacaagcactatttatcaacaaaggtaattttattccttctttcttatcattcctcctttcttatcattgtatattttctgatcacacttctctttgcaatacataatattaatcatgggtattcaaattcttgcatctttgcgaggtgtggcaaacaattaaaaattcagttaaatatacttgtaatagcacactaaagacaggtgctaagtttcaaggatgtttaatctattggaatttcctgagctagttatttaaaaattattattttgttaaacagattatccttcatttaaatgaactcaatgataaataattttgataaaatgtcaaaattagtttattttagtacagcatatattttaatttagtacctactggggaagtataatggtatgacttacctttatctgtatgtataggaataaagtagagacaatgatgtggaaatcaatagcttctgaagattccgtagaatataccagataaggaattccaaagttgagatggtgttgttacattgtgaaaagttgccaaacactccctctggggtgtattataataattactaccatcactgataattgtactagatgctttccatgctcagtttagtcctaaaaacaatcatggggaagaaaaaaaattttttttgtttttatgtttttatcctcatgtcttaattagaactattcatcagaattaatcactttgcgcccctcctcaactagaatggagtatacttccctgccttttttatgttgggcttgaccagtagaatgttaacagacatgtgcagaagctttgaataggctgttgtgatttgacttagtttttatgctcccctgacctataggagaagagaaaaatgtatggagcagaccaaagcatagctgcccagctgactcacagatttgtgagggaggaaatagatgcttataagccataagactgggggaagtttattatgcagcattgttacatggagttattagacctaattttgacagataagaaaactgaaacttttctttttttttttttttaattaatttattttttttattatactttaagttttagggtacatttgcacattgtgcaggttagttacatatgtatacatttgccgtgctggtgtgctgcacccactaactcgtcatctagcattaggtatatctcccaatgctatccctccccactcccaccaccccacaacagtccccagagtgtgatattccccttcctgtgtccatgtgatctcattgttcatttcccacctatgagtgagaatatgcggtgtttggttttttgttcttacgatagtttactgagaatgatgatttccaatttcatccatgtccctacaaaggacgtgaactcatcattttttatggctgcatagtattccatggtgtatatgtgccacattttcttaatccagtctatcattgttggacatttgggttggttccaagtctttgctattgtgaataatgccgcaataaacatacgtgtgcatgtgtctttatagcagcatgatttatagtcatttgggtatatacccagtaatgggatggctgggtcaaatggtatttctagttctagatccctgaggaatcgccacactgacttccacaatggttgaactagtttacagtcccaccaacagtgtaaaagtgttcctgtttctccacatcctctccagcacctgttgtttcctgactttttaatgattgccattctaactggtgtgagatggtatctcattgtggttttgatttgcatttctctgatggccagtgatgatgagcattttttcatgtgtcttttggctgcataaatgtcttcttttgagaagtgtctgttcatgtccttcgcccactttttgatggggttgtttgtttttttcttgtaaatttgtttgagttcattgtagattctggatattagccctttgtcagatgagtaggttgcaaaaattttctcccattttgtaggttgcctgttcactctgatggtagtttcttttgctgtgcagaagctctttattttaattagatcccatttgtcaattttgtcttttgttgctattgcttttggtgttttggacatgaagtccttgcccatgcctatgtcctgaatggtaatgcctaggttttcttctagggtttttatggttttaggtctaacgtttaaatctttaatccatcttgaattgatttttgtataaggtgtaaggaagggatccagtttcagctttctacatatggctagccagttttcccagcaccatttattaaatagggaatcctttccccatttcttgtttttctcaggtttgtcaaagatcagatagttgtaggtatgcggcattatttctgagggctctgttctgttccattgatctatatctctgttttggtaccagtaccatgctgttttggttactgtagccttgtagtatagtttgaagtcaggtagcgtgatgcctccagctttgttcttttggcttaggattgacttggcgatgcgggctcttttttggttccctatgaactttaaagtagttttttcgaattctgtgaagaaagtcattggtagcttgatggggatggcattgaatctgtaaattaccttgggcagtatggccattttcacaatattgattcttcctacccatgagcatggaatgttcttccatttgtttgtatcctcttttatttccttgagcagtggtttgtagttctccttgaagaggtccttcacatcccttgtaagttggattcctaggtattttattctctttgaagcaattatgaatgggagttcacttatgatttggctctctgtttgtgtgttgttggtgtataagaatgcttgtgatttttgcacattgattttgtatcttgagactttgctgaagttgcttatcagcttaaggagattttaggctgagacaatggggttttctagatatacaatcatgtcgtctgcaaacagggacagtttgacttcctcttttcctaattgaataccctttatttccttctcctgcctaattgccctggccagaacttccaacactatgttgaataggagtggtgagagaggacatccctgtcttgtgccagttttcaaagggaatgcttccagtttttgcccattcagtatgatattggctgtgggtttgtcatagatagctcttatcattttgaaatacgtcccatcaatacctaatttattgagagtttttagcatgaagggttgttgaattttgtcaaaggctttttctgcatctattgagataatcatgtggtttttgtctttggctctgtttatatgctggattacatttattgatttgcgtatattgaaccagccttgcatcccagggatgaagcccacttgatcatggtggataagctttttgatgtgctgctggattcggtttgccagtattttattgaggatttttgcatcaatgttcatcaagaatattggtctaaaattctctttttttgttgagtctctgcccggctttggtatcagaatgatgctggcctcataaaatgagttagggaggattccctctttttctattgattggaatagtttcagaaggaatggtaccagctcctccttgtacctctggtagaattcggctgtgaatccatctggtcctggactttttttggttggtaagctattaattattgcctcaatatcagagcctgttattggtctattcagagattcaacttcttcctggtttagtcttgggagagtgtatgtgtcaaggaatttatccatttcttctagattttctagtttatttgtgtagaggtgtttattctctgatggtagtttgtatttcagtgggatcggtggtgatatcccctttatcgttttttattgtgtctatttcattcttctctcttttcttctttattagtcttgctagtggtctatcaattttgttgaccttttcaaaaaaccagctcctggattcattgattttttgaagggttttttgtgtctgtatctcctgcagttctgctctgatcttagttatttcttgccttctgttagcttttgaatgtgtttgctcttgcttctctagttctcttaattgtgatgttagggtgtcaattttagatctttcctgctttctcttgtgggcatttagtgctataaatttccctctacacattgctttaaacatgtcccagagattctggtatgtcgtgtctttgttctcgttggtttcaaagaacatctttatttctgccttcatttcgttatgtacccagtagtcattcaggagcaggttgttcagtttccatgtagttgagcggctttgagtgagtttcttaatcctgagttctagtttgattgcactgtggtctgagagatagtttgttataatttgtgttcttttacatttgctgaggagagctttacttccaagtatgtggtcaattttggaataggtgtggtgtggtgctgaaaaaaatgtatattctgttgatttggggtggagagttctgtagatgtctattaggtccgcttggtgcagagctgagttcaattcctgggtatccttgttgactttctgtctcgttgatctgtctaatgttgacagtggggtgttaaagtctcccattattaatgtgtgggagtctaagtctctttgtaggtcacataggacttgctttatgaatctgggtgctcctgtattgggtgcatatatatttaggctagttagctcttcttgttgaattgatccctttaccattatgtaatggccttctttgtctcttttgatctttgttggtttaaagtctgttttatcagaaactaggattgcaacccctgcctttttttgttttccatttgcttggtagatcttcctccatccttttattttgagcctatgtgtgtctctgcacgtgagatgggtttcctgaatacagcatactggtgggtcttgactctttatccaatttgccagtctgtgtcttttaattggagaatttagtccatttacatttaaagttaatattgttatgtgtgaatttgatcctgtcattatgatgttagctgctgattttcctcgttagttgacgcagtttcttcctagtctcgacggtctttacattttggcatgattttgcagcagctggtaccggttgttcctttccatgtttagtgcttccttcaggagctcttttagggcaggcctggtggtgacaaaatctctcagcatttgcttgtctgtaaagtatttaatttctccttcacttatgaagcttagtttggctggatatgaaattctgggttgaaaattcttttctttaagaatgttgaatattggcccccactctcttctggcttgtagggtttctgccaagagatccgctgttggtctgatgggcttccctttgagggtaacccgacctttctctctggctgcccttaacattttttccttcatttcaactttggtgaatctgacaattatgtgtcttggagttgctcttctcgaggagtatctttgtggcgttctctgtatttcctgaatctgaacgttggcctgccttgctagattggggaagttctcctggataatatcctgcagagtgttttccaacttggttccattctccccatcactttcaggtacaccaatcagacgtagatttggtcttttcacatagtcccatatttcttggaggctttgctcatttctttttattcttttttctctaaacttcccttctcgcttcatttcattcatttcatcttccattgctgataccctttcttccagttgatcgcatcggctcctgaggcttctgcattcttcacgtagttctcgagccttggttttcagctccatcagctcctttaagtacttctctgtattggttattctagttatacattcttctcaatttttttcaaagtttttaacttctttgcctttggtttgaatgtcctcccgtagctcagagtaatttgatcttctgaagccttcttctctcagctcatcaaagtcattctccatccagctttgttccgttgctggtgaggaactgcgttcctttgtaggaggagaggcactctgcgttttagagtttccagtttttctgttctgttttttccccatctttgtggttttatctacttttggtctttgatgatggtgatgtacagatgggttttcggtgtggatgtcctttctgtttgttagttttccttctaacagacaggaccctcagctgcaggtctgttggagtaccctgccttgtgaggtgtcagtgtgcccctgctgcggggtgcctcccagttaggctgctcgggggtcaggggtcagggacccacttgaggaggcagtctgccggttctcagatctccagctgcgtgctgggagaaccactgctctcttcaaagctgtcagacagggacattgaagtctgcagaggttactgctgtctttttgtttgtctgtgccctgcccccagaggtggagcctacagaggcaggcaggcctccttgaactgtggtgggctccatgcagttcgagcttcccggctgctttgtttacctaagcaagcctgggcaatggcgggcgcccctcccccagcctcgctgccgccttgcagtttgatctcagactgctgggctagcaatcagcgagattccgtgggcgtaggaccctccgagccaggtgtgggatatagtctcgtggtgcactgttttttaagccggtctgaaaagcgcaatattcgggtgggagtgacccgattttccaggtgtgtccgtcacccctttctttgactcagaaagggaactccctgacaccttgcgcttcccaggtgaggcaatgcctcgccctgcttcggctcgcgcacggtgcgcgcacccactagcctgcgcccactgtctggcactccctagtgagatgaacccggtacctcagatggaaatgcagaaatcacccgtcttctgcgtcgctcatgctgggagctgtagaccggagctgttcctattcggccatcttggctcctacccgaaacttttctttttttaagagaggatctcgcttcgtcacccaggctgaagtacagtggcataatcatagctcactgtaaccttgaactctggggctcaagcagtactcctgcctcaatctcctgagttgttaggaggactacaggcacatgccatcacgcctgactaattaaaaaaaattttttgtagagacggggtctcgctgtgttgcccaggctggtcttgaactcctggcctcaggcagttctgtcacctcaggctcccaaagtgctgggattacaagtatgggctactgcaactggcctggaaaaccaaaattgttaacagagatgtgaaataatttacccatacaaaccacccaatatctaatgtgtatagctgacctctaatgtccctagctccattttttccaggctatataattttaaaaataacagactatactgattctacttttgatcttggctgtttatccaatgaatgtctttctgtgacatcttcaaccctttcctcattattttcttaggataaagtcctagagtagaaattctagatctaatatgcacattttagatttttgttatatattacaaagttatccttcataaggataagcagtatacctgatttctcatatcttttcataaataggaataacaataataatggcatctgtttcagttagagatggctggctaatagtagcttaaacaaatagaggaattatctgtccatatctataagtctagagcctctaaaattctcttggtatttcctgtgttacagtcaaggctagaaggaataatagtgtgatctagcaggcttctagttttgtgacagtggccagcagattcccaaatataagagaatctggggaagtaaggttttactattgttatttagcttttctagcctctataatagagattgcaaaagagaaggggtttgggaatgggtgtcaggtcagcttacctatagtgcctgccatagcagctaacattttttgatgtgcttgattgagcaggccctatgcgaagcactttaccaacatttaattcttaaaacaagttgagtagatcttgttcttcctgtttttccagcaaaaacattgaggttttgagagacttactaattttcccaatatcacatagttattaagtgggggagatgaacctgaggagtctaccccaaaacctcattcattaatttttagtgttcgtaatattcagaaactgaaagctattcaactccattagaggtcgtttctttgattactagtggggttaaacatctttccatatgtatattggttctttttagttgtattcttacttcttcttatttgtgtctttcatatatgttcctgatgatgttgtctttttctgtagctgttctttatagtttgaagaatattaaaccttcatcatatatatttcaaatatttttcctgacttgtaatttgccttttaactttatattcatgatgtactccctcaataaattagtacttaatgtataaatagacagatgtcaaaatctgttttccttagggcatctgttttttatgttataagtagcccaagattatgggaatatttaactgtatttttgtctatttaatgtttaaattttttcactaaaatgaatttattttagtatgaggtatgaattagacatctaacttacatttttccacaatgattaaccaattgtcccaatatcccttattgaattacccattactttaaaaatcccatcttaattatatattaaattctaataaagaactgctgtctcaacccttttcccttggtggcagtgtaacatagttgttgagagcatgaacatcagtttgagattaaacctcatctatactgcttattagctgtgggatcttgagttaattacttgacttctaaatgcctttgtttccttatctacaaaatgggaggcaataacagtaccacctcatagacttgtgaagcttaaatgaattgatatacataaactatttggaacaatgcatgttatacagaaagaaaccagtaaaaattggctattattattattttttaattttataatgaaaaatagtatttgttgtattgtgtccataccatacaaactgccttagtaataatgccttattcattaaagaaaatataatctttgaacagaagtggtatgtaattaaagttcaggtaacctttatataccattaattttgtaaagttcattattcatactagattcttgttttttatgtttacttttgataataggtagacattataacatctaagttctaaaatatcacagattatttttattttattgaaatatatggagtgggtgcagtggctcacacctgtagtcccagaatttggggacactgaggtgtgcagattgcttgagcccaagagtttgaaaccagccatggcaccatggcaaaaccccatttctacaaaaaatacaaatattagcccagcatggtggcgtgtgcctgtagtcccagctattcaagaggctgaggtgagaggatcacttgagcttgggagattcaaggctgcagtgagctgtcattgcgccactgcactccagcctgggtgacggggagatcgtgtcttaaaattttttttttttaacatatggaaattatattaaaccgtttgtagcccagtaattgtatcctttaaaatggaatttttaaatttactcatgagttcagaaactgttatttaaaagtcacaatttgtagagtattttgccaaggcaatagaaacaatgaggtggtttcttcctgcccaatatttataatttaatttgggacagatgctgatgagagtatagatgcttcctgtatgttatagtgtgaaaacaggatactgtctgtaaggaatacaagcagtttctctatgccagtaggaaaaaaaaatgctttatttaaaaatagtaaggagaccaggtgcctgcctgtaatcccagcactttgggaggcttaggcgagaggatcgcttgagcccaggaattcaagaccagcctgggcaacatagtaagatctcatctctgctaaaaataagaaaattagctggttgtggtggtgcacgcctgtagtcctagctacttgggacactgaggtgagagaatccctctgagcccaggagtttgagtttacagtgagctaagatctgcactccaggatggacaagagagggagaccctgtctcaaaaaataaataaataaatatgtacatatgtaaaataaaaatagtaaggatagttagactaattagatgctaaagataccaacttttaaatttatttcagtgtcattgtggaaaattttgaagcttttgggtttttgttaaacttataaatctcacttacacgcagcgtttttgaactcaaagtttagtgaagtatagatgcatcctcagttttctaatggttttcttctgacataggaagagaacctgaactattgttaactttgtttaccgattacatctgaattgcattcctctgttgttcaatgagcagtgttttgtgggatatgcttagataaataaattcatgtaaaaattacttatagttcaattaaatgtttgatttggtagccaaagagtatggaatcatagtcttgatcagtgtgaaattataggttagcgtcatcaacataaaaaccaagattctaagtcatccttgaacttcaaggtaattttcagagacccttgagattatgtgttagagatagggatgaaaaattgattttatcttttattccaacccaaatttagtagcagtaaatgcctgcagcaccatggtaagaaggactgcaaagctttcaggcttttcaggaaagaacactctagtactggctaccttggagtttaaggagacttacttttgaccattttgagggccttagcacagaactactcttggtcctagctggttagacaagcctagcttttctatgatcctccaaatgggatctgaataatccagttatcatgttagcattgaagataaagaactagtatattatatttattgggtctactaaaatttcatagacgggtagaattgactcttcagattccagaacaacccttcaggtcttggatatacaaactcctttagtgtagtgtccttgtgagcattgtctgtgggcgccaactttcaagtagttggcttgcagctcacaccagaatggaaaggacatgtttctaggaccctgaagagaattttcattgttcactgtttttatgcaaccaacaggatagtatgataattgtgtgtgttcatttaatccgtatttattgatcactcgtcttacacagtgtacttaggaatacagagataaatagaacacaggccctactcatgaaactcataatttgatagacatggcagtatcaataatttttgagtttgggcactacatagtcctcatgcaattgtttggctttcagcaagtcactttgagcaccagtttctttaaatgggtctaatggcaacattgctggttgagataatgtatgtgatatgtctcacttagtgtctgatacatggtagatgataactatcagtagcttacattttctagtacttttaaggtttacattgcagtttgacaagtaaaattgtattaaattcttatagtgtccctataagcttatattttttactttttcataaaccaagttaactggggtccagatatgttaagtttcttaagttcaagattgccaatcacgtcctaaaacttgtatttattcatacagctattccaacatgtaaatataaatttgttcaaaagaaatgagtgataagatatgaaatgagatggctttaaggaatgccgtagcacaacagaaaatcgtcaaatattgatgcctatgtggagggaagacaaagccaatgaactatgtttgtattaggcactgagtgatccaagcctttttattgttcttgacttagtccaatgagcagcaccagtgcctgcagtaatcagctgtttgtattatctaggagcccacttatagaattgggtgctgagatatcttattttgcattctatttagtagcctatgtatgtttggttagaaggagggaggagggagttgaaaggggagtttggatttcaagtttggcagtagtcattcacagtgagcaattttatatgccattattagaaatggaaatcagtcttgtagccatttagatcatgtgcaacaaaggcttttgaatatttttagttggttagttacttgctaaaattatgcaagaaatatgattttccctttatcttttttcacttttgggcttcttccattttgccttcaaggataacatataggtcatttctggaggaagaatattatatttgatagcttgatccaatgtggtaaactttaataaatactactgccccacttcttctatcaccctctcactcctgctattatccaggagaaatgtgatataatttctttcattagaattgaagggtgtttttatagtctttccattttttcatttattctcaaacattaggctgtgtaggtttgtaggttttctggccagttttgattattaagaatcacagcttttctaccatttaaggtcacatttatgagtgattcactaataaatctaagaactgcagtggcttgggagtaaatataagagaaatgtttctactgaaaagagaaacactgagaggcagaagtggaaggctatctggagggttgtggaattggcaatggtcagtgtttctgatccttaggtttgcaagcttataagcaattgaaaaagacagttattgaagacttaattttttctgaaagtactactgtttgattctatatgagcataattaatgatcatgctgaattaggaatttggtttgagggtttctataagaaacactgttggatactgcatttcaaaaatgatagaattttttcttaaatcttcacctcctactttctggatgctttttctttgataatatatctttatttgacccagttatcactagagttcagttgctaccagacttttcctaccagttgttgttggcatctgattccatctgtttactcatttattcatttcccgtaaatttttactccaaatatcccataggcagtgtgtcagaatatttttttttaaccagttgactttacatggcatttctttcagaacattctgccattcatttgtcaagtatttgttgaaagcttactgtgtgccaagcacagtaataggctatgaaacaaatgatcagtgaagttcaatccttatgtctaggaactcacaaattgggaaatttgggggatgaaggggagagaggttaagaaacataaagagacatataagcaaacaataacaatacatgttacctcttttttcaaagcacacttcataacttttctgttctctagtatctagcctttgtaatctttcttctgtactgttgtcagagatatttttcttagatgcagatctgatccaagttattctctgcatagtatacctatggaataagaaccaaacttcttagcatagcatgctggatatactgtttgctctccaaattctctctttaccatactctgttcttggggaggcagacctttatggattatattagctgagctcccttgccctttggtttcctgttgggtttagccaatgggatacggctggagattgcaaactggaaagaaagagaggtcagattatttattctcttggttctctacttgtagggtcattggttgacagtgactgcatcttcctgtatagctacagttgcagccactgtagctgccactgagtgccaataactcttgctctccagagacggattaaacgttaagataatgaaatttaaacttcagggcccctcacttgcaggggacttgcagaggccttaggaatctgtttacaaagctatttatttttgtaacatttgcaaaagttatttttacattctttctgaagaagggccgacggctgggcacagtggcttatgcttgtaatcccagcatttttggaggccgaggtgggtggatcacctgaggtcaggagttcgagaccagcctggctaacatggtgaaaccctgtctctaccccaaataccaaaattagctgggtgttgtggcatatgcctgcctgtaatcccagctattcaggaagctgaggcacgagaatcgcttgaacccaggaggcggaggttgcagtgagccaaaatcacgccagtgcactccagcctgggtgacagaatgagactccatctcaaaaaaaaactggggggggcgggtactaacaaaatggtataatcttcaggccctataaaactggaccctccaatgtccttaaccttgacccttcaagcttaggtaagtataaggtttacagggaagagagactactgaataacatacttgggaaggctattaatgaatatttcatggatgaaataataatttgagttggtgttgtaggatgaggagttcttcaggtgaagaaggatagaaaggtcattacaaatagaagacacagcctgttcaaagggaatgagtattttgatgtctacagtgaagcatactaggtagaaaacaaagaaaatacaaaagtcctgcggcaggaatatgtctgtcagttttgagaacagcatagagatcaatgtggctgtagacaaatgagtgatggggagaatagtaggtaaggttagagtttcctgttacttagggtcttgtaagccgttgtaaggactttgaccttttatcctgagtgagactgggaaacaggaaggttttgagctatgtggacatgatctgactattgttttaaaacaagtagtctggccactttgatgagaatagattggctgtgttgccacccaaatctcatctttaattgtagctcccataattcccatgtgctggggggggacctggtgggagataattgaatcatgggggtggcttcccccatactgttcttgtggtagcaaataagtctcatgagagctgatgattttataaggggagatctgatgatttctccttttgcttgattctgattttctcttgtctgctgccatgtaagatatacctttcaccttctgccatgattgtgaggcctccccagctacttggaactgtgagttcattaaacttcttttgtaagttgcccagtctcaggtatgtctttatcagcaacgtgaaaatggactaatacacagagagaccagttagaaggctattctagtaatttacacaagagatgataatgatttggacaagagagttgatggtagagttggtgagaaatggaaagtacagtattcaggatttgttgatggattcgatgtagggtattagagtgacagaagcgagtcaaggataactctagtatttttgtcctaagtaattgcaatggcaaattgctgtttactgagatggatgagactgggaagagcaagtttgaggaatggtgaaaatcaggagtttttttgtacgtgttaagtttaaggtgctatgttaatctgttctttcattgctgtaaagaaatatctgaggcagggtaatttataaagaaaagaggtttaattggctcatggttctgcaggctgtagaggaagcatgatgctagcatctgctcaacttctggggaggcctcaggaaacttacaatcgtggcagcaggtgaagggggagcccgcacctcacatggccagagcaggaggaaaagagagagtggggagatgctacacacttttaaacaaccagatcttaggggaactcactcactccctatcacaagaatagcaccaagaggatggtgctaaaccattcatgacaaactgtccccacaatccaattacctcccaccaggccccatttccaacactggggattacaatttgacatgagatttggtggggacacagatctaaaccatattattctgcccctggcccctcacacctcatgatcctttcacattgcgaaatacaatcatgccttcccaacagtccttcaaagtcttaacttattccaacattaactcaatagttcaaagtctcatctgagacaaggcaagccccttccacctatgagcctgtaaaataaaaaattagttagttactcccaagattcgatgggggtatagtcattgggtaaatactcctgttccaaaagggagaaattggccaaaagaaaggggctacaggccccatgcaagccccaaacccagcaggttactcattaagtcttaaaaccccaaaatttgactccatgtctcatgtccagggcacacgggggtgggctcccaaggccttgggcagctcagaccctgtggctttgcagggttcagcccccacaactgctctcatgggctgacattgagtgcctgcagcttttcctggtgtaccatgcaggttactggtggatctaccactttggggtctggaggactgtggccctcttctcacagctccagtaggcagtgccccagtgggggctctctgtgggagcttcaaccctgcatttcccttccacactattctagtagagttctccatgagggctccattagcagcaagcttctgcctggacatccaggcttttccatacatcctctgaaatctaggcagaggctcttaagcctcaactcttgcactgtgtgcacctgcttacagcttgcaccctctgaagcagcctcagctatacctgtgcccctttgagccatggctggaactagagcagctggaatgcagggagcagtgtcttgaggctactcagggtggcaggcactgggcgtagcccaccaaactattcttccctcctacgtctccaggcctgtgatgggaggggctacctccaaggtctttgaaatgccttcaaagccttttccccattttcttggtgaatgcaaatttctgcagcctgcttgaattcctcccctgaaaatagacttttcttttctatcacatggccaggctgcaaattttccaaacatgtatgccctgcttccctattaaatatgttccaattttatgtcatttctttgctcacacatatgagcataggttgttagaagcagccaggccagatcttgaactctttgctgcttagaaatttcttctgggttgggcatggtggctcatgcctataatctcagcactttggtaggccgagttgggtggatcacaaggtcaggagttcgagatcagcctggccaatatggtgaaaccctgtctctactaaaaatacaaaaattagctgggtgtggtgatgggtgcctgtaatcctagctactcagaaggctgaggcaggaaaattgcttgaaactggatagcagaggttgcagtgagccacgatcataccactgcaatccagcttgggcaacaagagtgaactctgtctcaaaaaaaagaaaaaaagaaatttcttcttccaggtaccctaaactatcactctcgagttcagagtttcacagatctctagggccagggcacaatgcagccaggttgtttgctaaggcataacaaaagtgactttttgcttcacctcccaatacattcctgatttccatctgagacttccttagcctgggcttcattgtccatatcactataagcatcttgatcacaaccattcaacaagtctctaggaagtttcaaattttccctcatcttcctgtcttcttctgagccctccaaactttccctctgcctattacccagttccaaagttacttccacattttcagacaccttacagcaacactgctttcctggtaccaattttctgtagttagtctgttctcgaattgctataaagaaacacctaagactgggtaatttataaaggaaagtttaattgtctcattgttctagaggctgtacaggaagcatgatactggcatctgcttggcttctgtggaggcctcaggaaacttagaatcatggcagaaggtgaaggcggaaccagcacttcatatggctggagcaggaagaagagagagagggaggaggtgctacagtcttttaaacagttagatctcaggataactcactcactcattatcacaagaacagcaccaaagggatggtgctaaatctgtcacgagaaactgtttacatgatacagtcacctcccaccaggtactgcctccaacactggggattacaattcagtatgagatttggtggggcacagatccaaagcacatcaggtgcctatttgacattcaaatgaagaaggtgaatagacaattggctatataagtctgggtagagtgggttgggagtacaaatggagtgttgtaagcatatagatggtgtctaaagccatatgactagatgagatactaaggaagtgaatatagatttttaaagggggagaaagaaagtgccaacatctgaggtttgggaccctccaacacatcagggaagtaggaagaactgacaagttaaagaagcagccagagagaaacagagaaaaaacagaaatatggtgatacagagagctaagtgaatgaagtgtttcagtgaggcagaggttgtcaacaattcttggtatatcaaataagataagtattgataattgaccgttggatttagcaatgttcaggtcattggtgatcttgatgatgctcagcagagtgaatttaaaatgaagtgagttcatgggaggagaggaattggaggcaatgagaagagacaacccattaggagttttgctgtaatgggggacagaaagttgttctttgggaaaagaggagttgagaagtttttgtgttttgttttaattattagtgttttaagatggaataaataatagtcatgtttgtatactgatgggaatgatccatcagagaaagaaaaattgctggagcaatgtctttgtccagtcaaggggggatgggatttagtgcataagtggagaggctggccttagataggaacatagacaattcatctgttatgacagaagggaaggtgtattatatggatataattcttgtacagtaggtgggaagatgtggtgggggtttttgaaaattattttcaaatttcttttttctcagtgaaatagaaagcaatgccataagttgaaagataggatagggaggtgttagaaaaaagggggaaaagtcatctaggagaatgagacagttaatacacaaggggaatgtagtatgatttctgggcagaattaaagccccacttgggattagtagtcatgaatttaaattgacatcagccagatatggtgtctcacacctggaatcccagcactttgggaggcggaagcaagtggatcacttgagatcagcctaggcaatatggtgacaacctgtctttatgaaaaatacaaaaattagccaggtgtggtagtgcatgcctctatagtttcagctgctaggaagactgaggtaggagtatcacttgagtctgggaggttgaggctgcagtgagccgtgatcacgccactgcactccagcctgggcaacagagacccctgtctcattaataatagtaataataataaagtgatatcagtcagcagccacattagctgcacagttgcaggtgcagaataagtagaaagttggcctttgctgagcaaataaaatgaagtcagatggaggaaagttgtcagtgtatacaagagaatgattgtgaaacatgaatatttccgattgcatttttcataatagccaaaagctggaaataacctaaatgttcatcaactaatgaatgaatatacaatggaatattagccataaaaggaaatgaagtactgatacatgccacagcatgaatgaactttgaaaacatcatgcttagtgaaaaaccagatgtaaaaggccacatatatgattccatttttatgtagtgtccataatgggcaaatccacagagaagataattagtgttatgattggggctgagtggaggaggaaaggggagtggctgttaataggaacatagtttctttttggagtgattaaaatattctggaattagatagtggtaatagttgcacaactctaaacatactaaaaatcactttagaaaggcagattttatggtatgtgaattatatctcaataaagctatataaaaataacatgctagctcactagaaatttgcttatcccaaactcaacaaattgaacagctcagaaatatagctgagctgtatttgtaatcaactaatgtaggactaaggtgaacaagtagctgtattacaatgtttgcagtctcttttcaggtttcaagattacagttgtttttttctcagacatcccttagtattaaaatgttattggctaagttgcagagcttgtgaggagagaccaattctggctcagtcttaattacttagtatcttcatctctccatcccttcctctccccttccaattaacaaacctttactaagctataaaaatcatcaagcactatcctaggtgctactggttatacaaagatggattggactttgtccctccccttgaatgtgaggtttaatggggaaatgaggtttaggaacttggagcacatttcatttttagggtgagactactctaatcgttcttcagcatcctcccatctatagcttatagataacgtatgcactcaaggcataagaaacttatttggatcttcattacgcttgaaacattcttccttttgtctctagaacatcagacattctttctcctcttactctaaagtattttggggctaccagatgaaaactcataataattttcttctgatgctctagacctgaaatatcttttataaaaacttcaacattcaaaattacgatgtatgttaggcaaagcgtgcatactggtgctatctgcaaaacaaataataatgtttaccttgcaggattgttgtgagggatcaatgagtatacataattgatatatggaagtgtcaaacacacgagctcttcaataaacattagtatactttatcactttgccaaagtctacaaacactaattttatatatggcaatatgttgagattgcagatatagacatagaccttaacagacaaaccctaattccaaagagtttgccattcattgatggaaattaattggttcagagatgttgaccatgtctaccttattatttaataacttaattaacttactacaaatctatcgatgttttccatcttggatttttatatcataaaaatgtagaattcttagctcatgactatatgaaaaatagatatttgataatgctttttaatgattataagctaattatattttgaatctcatgcctaactgaaatgtaatgttgcatgctggactttgaatttactaaaaagttcttttgttgtcttcctagaatggagctggtttgtcaaaatccaaaggaagccgaattggatttgatagcacacagtgggtatgtagaataaacaagaaatttctcaattataatgttcatttagttcattcatttactccgtaagtatttgttgaatgatggcaataataatagctaccttgtgtggtgggtggccggttggtagtggcaggtaagggacaggccctttaccaagtgctttatgcaatgtcttatttagtccctatagaaagtttaagaagtgagtaaatattgttactctcaattcacttagagagattaaacttagttggctgataatttggtaagaccagattctgtctgcctctaaaacccacattcactgagctatggtgtttccctaaatgaatgaatatatgaatcagatttatttgaataagggaaaagtaatgatcaggaataaaaatctattcaacctattcctttataagatgaggggaaaccagcaatatatacaatatatccttgttttgttttagaaatttcagaacctacacattgataaaatatattttcctatgttttaaaactaaatttagaaagaaaaacattgctgggttactaataaaacacaacatttattctgttagcatacattatgggaatgaccagatatttcttgatacacttcaatctttggcttctctataactagagatgtggaacactttaaattagaagtggattttcagatcaccaagcagtggtcattttagatcattgctaacaccaagtagattttgaactactgtttaaaagtaaagtctgggatatcctattatcaggctccccagctctctagtctataagtgtcaatgtaaacttttaatttattaaaaatagcaattgttttgctctgtgaatttagggtattctgaggataaaggtaagcatgatatacttggaagttatactacccagtcacagttataaagattttagattaaattaaaaagaggtattttgtatgcttctctgtaacacttctctacctccatcccacccttaggaaacacatacacctaatacttggacctgatttatcatcttgtggttgaagtaatttgctgagatttaaaattcagtattttaacagccaaaggcaacaggggtgatctttcatacattttaacattataagatgtgatgatacttagagaaacatatatttttcagatttgccatttattaggagtcttcatctgtacactgtaaagcaatttcagcaaaaaatttaaagccgtagtagcttcagttggataaaaggttttcctttatcggtattaaccaacaacattctgacaacattcccaaaccttttagtaaatagagagagcagtcagagaaagtacaggttcactgatacattttaaaatggaatttgtgaaaaatttaaagcttaaaataatagaaaaaagtagcgtgactctatccttttcattcaagaaatgatccttgaggtgggagaaaataatggatttttttcaaagtctttacttccacggtacgcaagcaaaaagttgaagagcagcttaccacattcagtgagttctctttatactcttttacattgaggggactaaaaaaaattgtaaatgtggtcactgaatgactatatttgcaaaatcacaggaaaggagaagtactaacatacttctaaacttttagaaggaataaaaggtgaaatctcatcaatagtgtgatattgagccctggtaaaattctagggctcaatgtttatggagttattaaacagatgacttgggagcacttagaaaagaaaatgatcataattaggaactaggcttttactaagaacaagtcctgccaagactttttaggttttaataaaattttaatacacaggcagatgaatgggctattatggtctcagcataatctcttttcaacaagatgtttttcagtcttataaacaaaatgagttactgaaggtcagatgataatagtgatttagaattaattggatttagaatcaactggacacgtttccaaggagcgttaatgattgtattgataacaacttggaggatgtgtttagaaggtgagttatagaatctctgcttgaccctgacctaatctgtatttatattaataatggtaatgaagctataagtgtgttcatcatatttgtatttaacaccaacctgagatccattcaacaaacattaaagtaccttttatgtagtagttctgttatctcatctttcttccaaaaccatttctttcttgtttttttcctagtataaagcacagaaagtaataaccctaaaagacacacacacacacacacacaaaatagctaaattggactattaaaattttaaacttctagtcatcaaaaaacactattaagaaaatgaataagcatgccacagagtagcaaatatttgtaaaacatgtatctcacaaaggaatggtatcaaagatatatgaagaactcccacacgactcagtaatagattttttgttcatgcctttcatcaagttgaggatgtattttattcctggtttgctgaaagttttaaatcatgaatagatactgaattttgtcaaatgcttttttctatattgaaattatcatagtttttcacttttttctgttgatttgtcaaattttattgattgattttcaaatgctaaagtaagctttcattcctaggataaatactacttggtcatgatatttactttccttttttatctttttttagttactggaattgattttctaatattttattaagtatttttgcatctgtgttcatgagggatggtggactatacttttttttgtaaggtctttgtcaggttttgctttttttttttttttttttgagatgaagtctctctgtcgcccaggctggagtgcagccatgtgatctcggctcactgcaacctccaccttgtgatctcggctcactgcaacctccacctcccgggttcaagtgattctcctgcctcagcctcctgagttgctgggactacaggcacacaccaccacgcccggctaatttttgtatttttagtagagacagggtttcaccatgttggccaggctggtcctgaactcctgacctcaggtgatccacctgccttgacctcccacagtgctgggattacaggcgtgagaagttttgctgttgagtatggcactggcctcttaaaatcagataggaagtattttctcctgctccattttctcagaaagtttttgtagaattggtattcttccttaaaaatgatagaattcaccagtgaactgtctaagtctgaagtttttccttgttgttttgagggcagtttttttttttcctaacaaattcagtttctttaataggtatagggcaattcagattttgtttcatcttgtggcagttttgttaaattgtatttttaaagaaatttgtgtcatctaagttgaattttttggtgtaacattgtttatcctaactttttacttagctgtttctcacactgaggtaataaacccctataaggcagagattattgtattcttggcatttgcataatactctacactaaaaacaaataatgagactgattcttagctttatctcatcctttatccttacaattgatattttgtctatttatttatcttgtatatatttttatgagttccttcagattttctgaataagaatttattcttaatttcatgaagcacctttttgataggcaaacattcctataagtcttgctttcattgaagtaggcttttaagcaatagtgtatgccagatattctgtttatccttgctgttcttagatattacttattcctaagtgtgatttagtccattttcattctactgttgaatttttgtttttttcagtaggggaccctacttactacccagcagagttatattttgaaatattgcggtattagaaaagcacattatatatggcagtcatcaagcaggcagtgtattttggtctgagtcttttgcttagaaagattattaagcagcattacagatatgaagaaaaatggtacaaacaactgaattttgtttttgaaagattaacaagactgatttttaaaagctgacggatagttctctcaattttgcttgaaaagatttagctaatactaagagaataattttttaagcaccacattttcatgtcagataccacttcctctgtgaaatttcttatccttttgatgtatggtaaatttgtagcttactggtctgtacttttataatatgttgtatatgtttttcttgtagcatatttcaccttatattgaaaatgttcatctttcttagaagactgcttattgagagcagagaccatatgtgctatttaatcatttgtattttttagcacaatgataagcatggtatctattgggtaactactctgcattcttatacaattaatgaattaaaatgttataaaatagactgttgtgttggcttactggaattacgagaattctttttctctcaaacagcgtgcagttaaaaaatttattatgttaacatccaaccaaaatgtaccagtgtttcttattgatcctttgatactggaattgattaataagaactttgaacaagtcaaaaatacttctcatggctctacttcacaatgcaagtttttctgtgttccaagagactttactgcatttgcactgcagtatcacctatggaagaatgaggtaagtgacttgctttcagataatggaatgtgtctctttttacaaaatagtataggtttaggctagtttaaaatgtaaaacattaaaaatttttcctgaaacactttataaattgtatcaggaatattttcagctataaataacaatacaactaatcactaaggcaaataggggatttctttttcttatataatgagaggttaaaaggttagtggctattgatattagtttagctagccactgatgtcaggacttgtgtctctgaaattctttattcatttacctcattatcacaggatagctgtcgtagctccacatatcacatccatgttcacaacaggaagatgagaggaaagattctgcttttttgctgggggaaacttctcaatatcggtatttttaggtcatttctgttgaactgtttgatatctcatagaaaaagcctacaaggcttatttttacaaagaatattttataatgtccctttatattccccaaatgaagttcatagaaattataaccctcctatatacataattccccaaatcaatataatgtattaactataatataacctagaaataaaaggaaatgatatgtattgctgtgtgcagatgctccagaatgactacactggaagacataataaagtaattcagatgcttgtatttagaagtaggatcacagaatgtggtagctacaaatataaacccatactatgaatgatattgttgttggcaatatgattttccaaaatagtgagcaagtttccaacaacaaaaaaagtaaaattgtctcttcattgacatgactattgtattcctgagaaataaaagctcagacaattataaacaagtttttcactatgtgattatgtgacaggacatttgaaattacatagtacacaggatagattttcatattttggattgtaggatatctaatgttcttggcctaggactctaaatgccagtttgtcattatgataaaccaaaaatatccccccaaatttctgaagtatctgttgggtacagtcccacttgccttgagaaccactattttagaagaaggggagtatgccaccattggcaaaactgatactaccatagtcaagaggaagaagcaaaagctcagccatacccagaatcagcacatgggttcaagtttattcttcgtttgtttttgtttgtttgtgttgggttttttgtttttgtttttgttttttgagacggagtctcgctgtgtcacccaggctggagtgcagtggtgcaatctctgttcactgcaatctccgcctcccaggctcaagggattctcctgcctcagcctcctgagtagctgggattacaggcgtgtgccaccacgtgtgactgatttttgtatttttttttagtagggacggggtttcaccatattggccaggctggtcttgaactcctgacctcaaatgatccacctgcctcagcctcccaaaagtttctccttttgtacatatgacatcctactattcaagagattcaagagcccttggatagtcccccctaaaacatcccccaatgtggagctaatcagattgttagatctaataatgaaagactccatttgcatgtgatttttctttattaatgccattaccataaagtgagcaaacctctgccaaggctactgggagtggacttttctagcaaaaccttgacctaggcctttacaccaattgatcagagcaactattttgttctttacttctcttgttgatggttataagaaagcaaaccatatcataattctgcctattttgtctgtcagtctttcctcctataacccaaggtcacgttcttctcaagttctggccggccttttaaatatttcctgaatttgtcagctgataatgcctttcttttattctattcagtagtgtctttctctgaattggctaccctccccctcagtcagtgctttctacttctaaggtgtaccaagaaagaaaagggaagaagggaatgttacagttgataatgaaacaaatgatgttggaaaatgaaccttgtcttacagtatgtttgttaatttctaatgatttgcattatgatggtgttctattatggtagtattttaagatgttgggatgtaaactatgagatgaaagaactacttttttgaagtacttttgaagataaaggttattaaaagttaaattaagaattacaagtttaattttaagtgctgtccttaaatcaacatttactttatagaaactaactggaaaacactaacatgagcattctcattccaaggaagggatttgtattaattttcatagagttttttttgttttttttttttgagacagggtctcactttgtcacccaggcttgagtgcagtggcacaatcttggctcactgcagccttgatctctcaggttcaagtgatcctcctggctcagacccccaagtagctgggactacaggtacatgccaccacaccttggcaaatttttgtttgtattttttgtagagacaggttgcccaggctggtctcaaactcctgagctcaagtgatccacctgcctcagcctcccaaagcgctgggattacaggggtgagctatggtgcccaacctataaagagagtctttggctatatctttcctgctacatactttgtatttttgctgctttcctttattctcccaccactaccttctgcccatcaccctcattaaaaaatgttcttacagagcagattagcacaaaaatatggctcaagttcaatataagaatcactttagttttgctactagtatttggctttaaatattcaatgtttaagtgttgtttcttgatgtttgatgcttctttggttctaggaaggctggtttcggatagctgagaatatgggatttcagtgcctaaagattgagagtaaagatccccggctagacgggatagactcactctctggaactgaaatccccctgcactatatctgcaaactggccactcatgcgatccacttggtagtctttcatgagaggagtggcaactacctctggcacggccacttgagacttaaagaacacattgacaggaaatttgttcccttccgaaagttacagtttggtcgttatccaggagcttttgacaggtaagttcagagtcaaaacgtgaaatgtgaaatgagtgttgttcagtcataattcttgcagtgtttttacatttgagtattgaaatctaatatataatttatataagtatttacagtaacattattcttaatgactccaaattagaagccacccaaatgtccttcaacaataaaaggattggctgggcactgtggctcatgcatgtaatcccagcactttgggaggccgaggtgggcagatcacctgaggtcaggagttcgagaccagcctggccaacatggtgaaacctcgtctctacaaaaaaatacaaaaattatccatgcattgtggtgggtgcctgtaatcccagctactggggaggctgaggaaggagaattgcttgagccctggaggtggaggttgtagtgagccgagattgtgataccacactctaggctgggcaacagagcaggactttgtctcaaaaaaaaaaaaaaaactgtaaaggaataaataatttttgatatatgtgttcatacaatgaagtattacacagcagggaaaaataaactaggggtctgtgcacattgtggatgaatcctacaatgctgaatgacacaaggcacaaaagaatctaaattctattattattattatttttttccattcaaaagtttcttttattcattaataaacaatgatatatatgtatacacagcttcataatcataccaaaaaagtttaagtgaactatcctttaaaggctgagaccataactttttgaacagaaataatatggattataagacagtatattgatttttgctgtctttattttaatataaagaacaaattgtgtggtaagactaatttattttcccactttgaaattaaacctctctagaaacatttagataaattatgaactaatctttaaaataccgtattacttcagcatttcaaaatcagtaagtttggaaactgtatttaagttaatattaggaataatataaccactgttgataactaacaatatagccaaaagaaaatgtggtacatacacacaatggagtactattcagccataaaaaagaatgagatcctgtcatttgcaacaacatggatagaactggagatcattatattaagtgaaataagccaggcacagaaagacaaactttccatgttctcacttatttgtgggagtgaaaaatgaaaataactgaactcatggagatagagagtagaatgatggttatcagaggctaggaagcatagtgggagaaagaggggaagagggggatggttaatgggtacaaaaaaatagttagaaataatgaataagactgagtatttgctaggacaacaaggtgactatagtaaaaaataattgtacattttaaaataactaaaagtatacttggattgtttaatacaaaggataaatgcttgaggtgatagataccccatttactctgatgtgattattatgcattgcatgcttgtatcaaaatattgcatgtaacccataagtatacacacctactatgtacctacaaaaattgaaaatacaaaagtgaaagtaaattctattattacttttataaaaagttcaaacacatgctaaattatgttcatggatgtatacccttatagtaaaagtattaagaaggctaagcaagacgtaccaaaaaagactagatagaggacacagagaactacagggaaactggaagaattttatttctgtggtggagactttggtgtttactttataattcattattttgtgcctttatgttatgcactttcctatatattttttaaaaccatgtgcaaaaatttatctttggctatctcaataataaaaatatttcttgtgagaaacagttatttgaaggaactcatgtaaaatttgattagctatagtttataatattaacaattacaggattaaaaacattcttgaagttatacttggagtatgaagtttctaacctagaattgttccttttattctccttttgaaatcagcgataatgatgttacagtctactttgaatagcagaatctgatgtaaaggtagcagtaaatatttgtaaggattttcacattaaaaactccttcttagtaacttccagtgagataattcttatctgttacacttgagaagtgtaagagtatgtttattcttgccttcttttaaaaatatatatatatattatatatatatgttttctctctctctatctggaatcatgtgagattgccttcttattagtacttaaagtcacatatttgagaatgactgaaaaaggtattcgaaactgaagtcttctatattttttgtgtatgaaaagtcggaacttttctgaaccaagccatattttcaaaatgaccaaaaaaaatgagtagagatggagaacaatactttgtttttattattggcttctcttattttaatcaaaaatcttaatactcactgttctcttaccacttttttgcctgtttttttcttattctgtatttcaaatgaccttctttagggagacattatcttttagttttttaaagctttgtgaatttatttcaaaatttaataacttagtaaagttcaaaattgtcagttacttattaaacataaacatgtgacaatagataaaagctatctctacattgtaaaattttatatgagtaggaatggaaaactctcaaataatatttttagagtatgggatccaaaatacataagatagatttgcagattagcattttacccattaatgagattctcaggccattgtaattaacttgtgtgtcttaagtgttaaaaacatttacttctctaaaagtaaactgataattaaaaattatgtcacaaaatttttgtttctgcttaaaatgccaagtgtgtatgaacaagtacaaatatattaatatataaatacattaaccaaaataattaaaactcaactgtttgatgtcagatttttcaaggtcttattaaaattgctaattgatatctgacataattgatgaaactatgcttgatgtttaggtattttgctaatgtttgatatttgtaagaggctgccagtattctgggttaaatccttttaataaatcttttattattattattattatttttaaattttactttaagtagtgggacacatgtactgaacgtgcaggtttgttacataggtatacatgtgccatggtagtttgctgcacctatcaacctgttatctaggttttaagctctgcacgcattaggtatttgtcctaatgttctccctccctgtttcccccacccctcattaataaatcttaacttttgttttcaggccagagttacagcaagttactgttgatggactggaagttctcattccaaaggatccaatgcactttgtagaagaagtaccacactctaggtttattgagtgtaggtataaagaagctcgagcattctttcaggttagagacaaccaaatgtgtacttttaaattaaagaaaatgttgggattatttttaatatttgagggtggtaagatgaaggggcttatggaaaatagaaaagtaaacatccttttttgatatgtctcttttcttctagattgttttctttcagttttttttagaagtagattaaaaattaaccttaagaaactattttctaagtcaataggttgatatttatttattgttttatttgaataactttaatagatttagcactggcttctgccttaagatagcccattaactttgtgaaaggtggtgtattctcagtccaagtaggataaagccactatagaagatggaccatgtagatttagaaaagacttcatgaaaatacagtttgtttcagagttggcattgaatataattttttttgcatttatgaaggtttttgaagataaatgctacacaaagaccaggtgcttttaaaactttattctcttgctgcagctttcaattcaatacacatttattgtgttccgcaggcttctggccctggggatataaagatgattttgaaaggcatgaaagttcagctctaagagatgacatgaaacacagagatacagtgaaaacaggcaaatttacagtggggttttggtacctgaattctttcacttgccctttattttctggggttccctgccaagaaagctgtgtccacgagggatacgaaaatgaagtatataactgtcaagtgcccaagacccacaaatctgaggtttctctaatacagtgtactggcacctaaagctgaggcctgacagcccaagtgggccttcgtagccctatttccttaagtcattgtggagctgtgaaatttatgcagccagcctcatgaataaaaagctgaaaaaccacatgtgtggatgggcctactctagtagaaaagtgctgcctgacatatgcctaccacataataacaggaagtagaagagatggagttttgtgcttaaacttgaccgctcttcctgtcctaagggagtttgctgtggttgtcatctctattatagcaattatcacagtgaattatgaatatctgtcttgtcctcttatcaagttttatgaacttcttgataacaggagtgttcttttatttacctgtgttggcccagtatctactgtacctggcataaagaaaagatccagtagggtcagttttcaaattaaagtgaacatacatgtatttgaacacttgatggcgccaaacagtcttaaatgtaatgcttggtgtaaagcaataaattaatctaatagacctcatcaagcagccgcctttctttttttaaaataatttttaaaaagcaattttaaatacataaaagctgcaagtacagtaccgataacttttttttttctgaaccacttgggagtaagatgttgaccacaacttcaaaaaatttagtatttttttaaaaataggaacattctctacatgtcctaatatgaaagttaggaaattagcacatacatttttaccatttaatccctattcaatttttgtcagttgtctcaataataacctttgtaataaaaagattcgattcagaatcacatgttgtcttaattttcctgtctctttagtcttcttcagtctgggacagtttctcagttcttttattactttcatgactaatactttggaagattacaagccagatgttttgtgcagtgtccctcatttggggtttgtccgggggttcctcatgttagatttaggttatacttctttagaaggtatagaagtggtgctgtgttctcattacatctcactgggcactgcataattttgatttatcccattactgttgatattcacattgttcacctgattaaagtgctgtctgaaacttcgtatctttaccactatgaagtttctgtttttccctttataataataagcatctggcaagaagttactttaaaactatgtaaatattgttttcctcattacattttcaatttatttgttcatatcaatataaataaattcatggtttcctattttaccctatgggttatagtcaattattttcattatttattttgatcttcagattgttccatatttggccagtagaaactccttcataatgctttctgtgtccttttgacttgtctccgttgttttttgaacactttagtactttttggcactataaaatattctgggttcatcttacaattttcatacctccaccctgggatcagccatttctttaagtcctgtttccttttagaagccaagacctggatgccaggtgtacccattgctatttgggttttgctgcagagagtttctctcagtgaacaggggtagggtgtatatgtctgtgtgtatttatttctgtatctatctattgaaacctctgaattcacattgacatctccagtccggttaaaagttccaattaaacaacagagttcatttccatatttgcgactcccttttcaaatcgtgagaaatctgactcccattgaccttaatgtttacttagttgttcagtctccctgtatgtaacctatcttccaacacatgtcctcccctccctaccccctgttcttctcaccctacctgggcactgctatcctctgctgggctgcacacacgtagaggcattcttcttaccctgttcaggctctgacttcccacacctggctgctgttctgcagagaggctttcctcaccctgcttgggctctgactccccacactggacactctcctactctcttcatgtggatgtcctcattacctgcctaggctctgataccccatatcaggcaatccctttgcacaaaaacctttcttgctctgccccatctaatggttttagtatcgaatagttcaggaagggcgggagactttatttacttttaattattttctcaatctaccatgaagttcaaaaactagaataatataccttttcctgaatttgattttgttttagcaaaaaccatcacaagataattaatgagctccaggctgttgaatatcagtgaaaaaccaaaaggaaagttggaaatacctgtacacctggcctaggaatatctagataacaatatttttattttatttctactaatttgctctaagattttgggcaaatttctgagccttggtttcctcatctacaataagagttggtaccttctgtcatcttattctttgatataaggtttgtgcttttggattccacgattcttcttgggctttgtgtccccgttcattggctgaacaggaaaaattaaataaacatgatatttaaagtaggatattaattttgtctttttttagaggtatagtaatcctgagatttgtacttgggatttatttttatttgtttacttatttattttatttttaacttgtaagttcaggggtacaagtgcaagtttgttacataggtaaacttgtgttgtgggggtttgttgtacagattatttcaccacccaagtattaagcctagtacctattagttatttttcctggtcctctttctcctcccaccctccaaaagaacccattgtgtgttgttcccctctatgcgtccatgtgttctcatcatttagctcccacttataaaaacatgaagtattaggttttctgttcctgtgttagtttgctaaagataatggccttcagctccatccatgtccctgcaaagaacatgatcttgttcttttttatggctgcatagtattccatggtgtatatatactacattttatttatccagtctatcattgatgagcatttagattgattccatgcctttgctattgtgaatagtgctgcagggaacacacacatgtatgtgtctttataagagaatgaatgatttatattcctttcagtatatacctgataatggaattgctgggtcaaacagtatttctgtctttaggtcattgaggaatcaccacactgtcttccacaatggttgaactaatttacactcccaccaaccgtgtataagtgttcctttttctccacaacctcaccaatatctggggtttattttattttattttattttattttattagtttttttttacttgttatagtagccactctgactggtattagatagtatcgtattgttttttattgcattttctaatgatcagtgatgttgaacttttttcatatgattgttggccacatgtatgtcttttgaaaagtgtctgttcgtgtccttcacccactttttaatggggttgtttggttttttccttgaaaatttgtttaagttcctgatagatgctggatattagacctaatagttaaggtttgcaaaccatagtttgcaaaaatgctctcccattccataggttatatgtttactctgttgatagtttcttttgctgtgcagaagctctttattttaattagatcctatttgtcagtttttgcttttgttgcaatttcttttggcatcttcatgaaatttttgcctgtgcctgtgtcctaaatggtattgcctgggttatcttccagggtttttatagttttgggttttacatttaagtctttaatctatcttgtacaggatatttttaaatgaaaaaagtatgtatactataatttttaaaatttatagcagatgtttaaggtatatagctctatgcatgtatgcactttaacacatacaaggatcagttctgagaaatggaatttctggctgggcgccatggctcacgcctgtaatcctagcactttgggaggccaaggcgggtggattgcctgagctcaggagtttgagaccagcctgggcaacatggcgaaaccccggctctacaaaacacacaaaaattagctggacatggtggtgtgcacttgtaatcccagctacttggaaggctgaggtagaagaatcacttgaacccaggaggtggaggttgcagtgagccaagatcatgcccctaaattccagcctgggcaacagagagaggagactttgtctccaaaaaaaaaaagaaatggaatttctgagagtgtcatgttaagaaaagtagattggggtgggaatatgtccatatgggagcagtaccagcagcaggtaactatcagacctgatgtttttgtagagcacaaatttttcatatttgctgtttagtcctttcagtcactctgtgtaataaggcaaggattcttttaacaggtaagaaaattgatgtttcaagatgtcagttacatggtcatcattggttgagcatggactaaatcctaggtctccacctcttaactccaggcttttcctactacaacaagcattataacatgtatctctcattccagtcatttattgtaagagcacttatggctttgaggaaagggatgtattcaaattgaagggatcctgtgtaatttgtatattctgtagacagtgacttatctgcaagaaattcttcttactgaaggtagggtactttttgcttaagattcatatagtccatccaggatctatattctttcctactatattgtaaaagaattacaggatattttaggatgttgcaggcctgggaggggcttagtcaatcatttattcatttgcccattcatcagtatgtgtttttcagatattatgtgccaggcaccattctaaacctgtagatacagtgatgaagagatgtagtacttgccctcagggaactatctttacagtctagtggagggaatataaaattgatgattaggaataaatatgatatgaattatagtaaaagtatttacaagtggtaactattataagcttgttaaggaaaaagataattcatttgtctttgtatatctagaaccaaacataattctttgctctataaatgttgaatagaaacacttcctgaataggaacattggaagaataaatacatatgtcttcctgggaaaactggggaatgttttgcagaggttggagctgagacttgaaagattttattgatcagggccatatcagacaaaggaaacaagtgcggaggcttgaaaagttgtggtgtatttgaggagttacaagttattgtggtatatttgggggtttacaagttataagatgaagtgtgaggagatgcagatgaggctggaccccagtagtcaggaaccagaacacagtgtttatgtccaccaggacaagaagtttagattttgtcccacaggtagcgaagcaacactatagaatttatagtgctttcctcagctccagaacactctaaaaacgaagagaatcagaaaaccaagatgactaaatgatatatatgacctgacaatttgcaagacatttttctccttcaatcttcacagcagtcctgtgaagtataataattatctttaaactacaaatgagaaaagtagatacaagagagatttgtttattacattctttcattcattcagcaaatactcaggcactactctacccactggagatataatgataaaatgaatgcactttcctcatagaaagtgaggatgatatgtacatggtcaaagctaaaaagaagtgcactagatttgataatctgattcaaaatctcaggctttttctactatactacacagtctctaaagaccaatagaatcactgaatggtgaaaacattattaaattctttttgtttcagctatgtttgtagctctcataattagctttattttatcctgattgtccagctactaaattgtgatgtaaaggagggagctgataaaaggatgtctcatcctttgggaatcctggttctattctttcccttttaatttatctctccaagaatctgctcttaagtgttcattttaatgtgggacaaacaagtaactgtaaaatgtggtttttataatataaaaagattatatggggttagttttcttttttttctcctttctttctttttttttttttcttttttgagacagtctcattctgtcgcccaggctggagtatagtggtgtgatctttgcttactgcaacctccacctcccgggttcaagtgattctcttgcctcaacctctcgagtagctggaactataggcgcgggccaccactctcagctaatttttatgtttttagtagagatggggttttgccatgtgggccaggccagttttgaactcctgaccccaagtgatccacctgccttggcttcccaaagttctggggttacaggcgtgagccactgtgcccagcctggggttaattttcaaatttaattcagatgccacagaaaggttcctagcaatttagaaatggctgtaatagctgactatttattatatctgtagcagtaccttgatgataacactgtggaagctgtggcctttcggaagagtgcaaaggaattactgcaactagcagcgaaaacattaaacaaattgggagtaccattctggctgagcagtggaacttgtctaggtaaaattcttacgactttccatttgtctttctgtcattttgtcctctggctttagggattactgcttgagatgacaaaatatcagtgacatttgaagtgtcatgtgtatagacagaataaacatgagtgcatgcagcaaggatctattgatttccttaaagaaattaatttgagaattataaaaaagaatgttagaaaggccatggttgtgtttactcataattataaataatatgtataaaatgtatatcagaacatgtagactatacaatagtccccccttatccatggacaatacattccaagaccaccagtggatgcctgaaatctccgatagtactgaaccctatatacgctgctctttccctatacatacatatgatgtttaatttataaattaggcacagtaagagatgaacaacaataaataataaaatggaacaattttaacaatactataataaaagttgtgtgtgatctctgtctctcagagtatcttattttactgtactcactgttattcttcttacgatggtgtgagatgataaaatgcctacatgatgagatgaagggagatgaaggatgtaggcattgtgatgtagtgttagtctactattgaaaatttcctgggaaaatcaaggaatgtgtcacagaggctaaatctgagccctgaaagatttgatttaacacttctgaattgtttatttctggaatttaccatttaatatcttcagatcgtggttgtccacaggtaactgaaactgctaaaagcaaaaccacggatatggcaggactactatagttgattctcagataatccttaaattagcattttattatttctatcccaaagattgttattgcctttttttataattataaaaaaccctctatttctttacttatataccattcaaacagcttgcattgcaccaaatgtttctactgagaggaacattaaagacagtgtcataaggtcttccatcagcctttcctaggtcattggtagtatcactaactagacatcactgttcatctgacatggacatacagacttttctacagtccttaagcaggttgctattagaatctgtgagtgatttctgggtctctgtccactgtccattaaatcaaacttctttggaatttagaattatttagaatcttaaattttgttttgtgtttatttgttgtctcttgattatcatgatagttaattatagctgtatttgctttttctttatagtaaccatatctgtacaaaagttaattcaactcctgcctttatagggatagggttgccatccaatttattgttcaattcaagagacttgagagtgaaaggaagcaccattaataattatgttggtacaacaggcataaactgggatatacggttatcctatctattagcctttgttgaaaatttacatggttcttcctgccaaggagcttactactagaataagccaaaaaaaaaaaaaaagtacatctcacacatttatgtgatatttgctttaaggtttaattttttagaaacaagattgttttataatgtgtgtcatcaaagacacttcatagtcatttgacatgatttgttttgagttttcagtcccatggttttctgtctgatttaagggcacttatgagggagttgtattagatgatatttaagaaaacttttatttttaattgtttataattctttaatagaattattttagaattccaaacaatattatccaacagcaatgcctataaggataatcgcagtcatttatttacttttgaaataattggaatgaaatgattagaaagatcataggggagacccaggagtccttaataatattaaggtacatgttttatttcttcagaacagtgctatagcaatgaattagagcacatacgtggtaaacacttagaaatatcatttggcagtgtgttgaacattgaagctgctactgcttttctttttcatacggcccatcaggtggtcactgttgagagctgttaggttctacaaattattgctcaagaaaaatatattggttaagcaaaagaattaaatattttttgcatatcttaacagccccctctatcactagagattaatgattaaacattcttatcagcaacttagtgttattaaagctaatggtttattcagaaactaaaatatatcatgaaagtttttgaggaagctgagagtgctcagacagtaaaaatagatacatagatagatagaaggttcaggtgactgctcaaacaaagtcatttagtttgaggtttaatttttaaaaataattttggtgaagcatcttaagtctaatcctgtgaaataaaatccattctatagccccagccactcaagaggccaaggcaggaggatcacttgagccaggagtttgcgtacagcctgggcaatatagtgagactctgtctctttaaaaaaaaagaaaaaaaatccttgttacaaatataatttgttataataactaattttttccaaacctaaattttgttaaaaaaatttaatcttctttttaggatggtatcgacaatgcaacattattccttatagcaaagatgttgacctaggaatttttatacaagattacaaatctgatattattttagcatttcaggatgcaggacttccgctcaaacacaaatttgggaaggtcagtaacaaaagtcggcttcatttcataagtaacatatctcacttgtaaagtttacattaagcaactcagatatggttaagaatgctacatacataattttatcactcagtattgactaggatgagttcagcagaagcctgttaccacttgtaatttctgcactgtctaggcaaaagcaagaaaatctggctttctactgggttggtgcaaaagtaattgtggtttttgccattacttttgcaccaataatgataagaaaagaaggatcttgaactcttataggtgaatgtattgctattatattaggcaacaatgtaatataaaatcaatataatgtataatatacaattaataagtaagaatcccacccgccgtacctgattgtttctcatgagtcatttaatttacagatgtcattatcaacataaaatattccattgattgctaagggatagaaatatagaatcatttcaaataagtacttcaatttcttgtttatcttatatgtcctaggctatagcagtttgctcagacatcaactagggataggtcattggggcctagatgaaatctccctctagacaatttgattcctatgccctaagcccatgatctcttgcaatcatcttgttcttaatttgcttgtcccctcggaggtgttaccctacaagcaagtaaaaatatgtttagtcggctgggcgcggtggctcacgcctgtaatcccagcactatgggaggccgaggcgggtggatcatgaggtcaggagatcgagaccacagtgaaaccccatctctactaaaaatacaaaaaaaattagccgggcgcggtggcgggcgcctgtagtcccagctactggggaggctgaggcaggagaatggcgtgaacctgggaggcggagcttgcagtgagctgagatcgcgccactgcactccagcctgggcgacagagcaagactccgtcttaaaaaaaaaaaaaaaaagtttagtcaccagaaaattattttttccatcataaatagttattttatgttactaaaaaatataaataaaatattttactgaggtcaaagtcaaataacagagctctagttattcagcaaacatttaccaaacattcactataagtatggcactgtcctctgcacctgggagacaaagatgaataaatgatagttcttacccttgagaagctcactgtctaattgggagggggaaaggctgcataaataattctgtgatgagtgctgtggcggacagatgtaccaagtccaatgggaacgtaattatttgtatgataagttttctttagggaaatgttctcagaattatttatttttttaccttaacttttatttttttcttttttccatgtgtgtagtataatgagctagactatttatgtatgtggctatgaggaatgccactttacttaagtacttattgattgttatgagagacttatttcctgatagttttatttggattattaaaggaaataatatttctttggttcttttccttttttagtcagaaagctgctctggaataggatatttctattttttttctgcagtgataattaccataagtcatttactctgagttatcatcaattgtaagaaacattattttagatgcagttaagaaattaaatgatatgttactgatgcatcccaatttcagaggtgccttaacttgaaaaaatgtgcatcttagaatgaatactctatgtatgtaaaacttaagaatctgtttctttatttttattttttaaaaaaaggtttttaaaaatgtatttcctttgtttcagtgtgtgaaggttttcatcttccccataggtagaagacagcttggaactatccttccagggaaaagatgatgtaaaacttgatgtttttttcttctatgaagaaactgatcacatgtggaatggaggcactcaggccaaaacaggaaaaaaattcaagtatgaatcaaataagtacttatttataaaggtactacagaaataatttcaggaggtagaaataaagaagtaactgaaaagaaaaccaaaaatctctttcaagactccattattagctaacactttcttagcttacccatagagtccagttatgcctgtgaagtaagaatacctgtaaggacggtttgtgaggaggaagtgtccctgggtttgtcagtccaagttgatgatacagctggtctattctcagttctgagagagagaatgagaatgagaacctgaagagcatgggttttagagtcaggctgacctgggaaaccttagctccaccctaatttgtggcctttagattttctgaacgtaatcattttatccattacattgagtaatactactgtgtgtcaggcactattctgaacgttttacatatattaacccatctagtcctcaaaataaccttcagaggtagatattctgaagccagtgtgattgctgttgaatctcagctctttattttaccagctatattaccttgagcaagttatttaacctctctgcctaagtttcctcagctgtaaaatggaaattatagtagaaattgccacatagagtggttttaaggattaaaagaattaatacacaaaaagagctttgaggtgtgtcaggaggtcctgggtgctaagtaattattacctgctgttactaatactactatagtagtagtagtagtagtagtagtagtagtagtagtagtagtagtaaagaaaactatttctcttcttattctcatgagaaatttacagattagagacatgtataattatctcaatattaaactgttacatctattcttagagaacttctgtaagagtgtcaccttttttctaagaaagataatttctagagccagtattagagtcctgttattcttaaattactttctaaggcttgaattttttctctcactgacatgatccgaaacctgcaaacctcaaaagaactgttcatttccaactactacatttctggagagaaaaagcttctttcattctgctttaacagctctttatagtagcagtgtttgggaagtgtgaagtgttctgattatttaacaagagaaatgagcagtgatagaactgtctggacagatggtgtgagtcccagattttctatcatgttactgtgaccttaaaaggcagagaaaagaacaggagatggctgagtagagtagtttctttggaagattcccccagccatatgccatttttattcttttcggcactatttactttaagaaaatgtagtatttttaacactactattccttggggatgaagaaaaacaaaatgtttaaagctagttcaagggtctttttaatgtattttaaatttttgaatagattatacattacatagttaaaatattcaaagaatataaaggatgtgtatgaaaagtaaacctttctccatcctctgcccctcattttcccgtttctagttgccctttacagagataaccatgattactcatttcttatgtatcctttccgagacaaacatatgctcgtatacatatagtatttacgttcatctctccccctttacacaaatagtattatggcatattacacactgtctgtatgttcttttcctcacatagctatgtatcttggaaaatgttccaaatgagtatgtatagaaatagctgcattttattccattgtatggcaataccataatttattcaaccaattccctattgatgaatatttaggctgtttccagtagtttactgtgaccctcagttctgcagtcactatctctgtccatatgtctttatgcacacgtgtgaaaccctgtgcaggataaagtattagactcaaattttggggctaaagggaatataagcatatttcaattttgatagatattgccaaattgccctccaaagatgtttccccaatttatattctcaaccacatggtttgagaatatgggtttattttttaaaagtgcactatctgtaaagagaggtaaacttgctcaatatttgccactaatcagtaacttatcaattacttgtaatcagtaactaaatctaccatacaccaaatataattgggagcacattagaattactgttcaaactagtcagtataatgtatcatctcaccttctccaaaggtctttttgtctttataataacctattttttattttatatatagttcattctgagaaaagcttaataatatagaatgcttactattttttaaaaggcagaagaggaactcaagaaggaagaaaaaagattttctttctaaactactctgcaggactatagaatgatatctttggtcctaagatttaacagtatattaagagtaataaaaaagataaagcttccaggatatctgctacctatcaggcactgtgataggtagttcatatatatatttatatatataatctggttaatcctcatactatccctgtgggttcggtattctcacctccagttagacattaggaaactaaagctcagagtgaagtaacttactcgaggcttttgactgttaatggcaagatcaagatttaatgccagacctgtttgacccctaagcctaaatgctttcttcttagagttaataggttaagtgagttagtacatctaatgcatttagaacagtacctggcacattgtaagtattgtgtaagtagtagctactgtcagtactgtattattattattactgttactgttattataattaccatgctgcactggcataaggtatggtactttcagcacagtggtaaattggattagtaattttctaggcaggcatattttcttcctccatctcatgatactcattccgtctttagttctcaatctttcacttctttataggaagcccttcttttacctgaaatccaaattccatttaaaaatattgactggattctttattctgtttttctccagcatccaaatctgccagtaataaaagtgatgaatataataactatgcctccagaatgtgaagttcttaattcaacttcacatttcctaaagatgctgcctagatttatttggtttgcttctttccttcccattttgaatcaactggtatgggtagaagccagaagtttgaaaggtaataataatagttaactttattgaatacttactataagccaatcaatatgccaagcttttatatgtgttatcttatttaatcctcacaataagtttataaaggagattttatcatcatcacctttattttatggatgagcaaattaaggcagacctgagtcagacctaggtgtgtatcacttcagagcccatgttcttactaagttagtgtcaccatgatctctatcatgttgttaataccccttccatgaaaacattatcagggtaatacaactactgctacatcctctaataggaaatctactccttgggctagtagtgggttccttataccttctgacagttgcagcttctgattattggatagatcttcagaaaattcagattcatcctctgtggaccacactcccatccaggtgtggatcctgtgtaatttatcacttcatttctgtaaaatgtatttaccaactgctatgtgctaaggatactgatgtgactgtaacttagtttctgctcttaaggatctcatgatctagaccatgagacatgttaaagtactctgatagcagtactgtaatcaaatatgtataatctatagttgaagtaccaaatcagccatatctagaaacaatggcaaagaagtgtggcttacaagtagagaaatttgttaggtagacttaggagaaatgtgggaaaagtcctaaaaatagatttatttaatgatttttaaattagtttatttctattttttaatttaaaaaattctgtgggcatctgtatacgtaaagtaaaaactttaaggggttgtttccttcaatagatacccaaaggtagaattattaagtcaaaagatatgagccttttaaagagttttgatacatattgccaggttgcattcctaaaaagttatgcaaaattttatacagtcaccaacataaatgagcatgcttagtttgctatatcatactgagtgttgcattgtactcacagtcattcatgactcccctgatagtttctttgagtaacttttcttttcactttcttcttattatcccaaggtatcttctatcataaaaccaggtcagtcattagtagcaagttaccaacaattattacctttctggccaggcacagtggctcatgcctttaatcccagcacttcgggaggccaaggtgagagaactgcttgagcacgggagtttgagaccagcttgggcaacagaataaaccctggctttatataaaaattttttaaaaattacccaggcatggtggcatgtgtctgtggtcccaactacatgggaggctgagacggtaggatcacctgagcccaggaaatctaggctgcagtgagccacatttgcaccactgtactccagcctaggtgacagagcaaaaccaaaaaaaaaaaaaaaaaagaaaaagaatcattacttttctcttaactattcctaacatcaactggcttttagtatacatctaaccccctccctgtcgtcccagtctccctttcaaaatccagctttaaaatattacagtgcattttgaatgtcttgttataggtgtttgttagacacttattatatagagacttttatatttaagctttatacaagtgtgattttagctgagtgagcccaggaattagaagacctgaattcaaatctgagttctatttttttgtgtcatataaccttctgagcttcagatttctcctcttaaaatgggaataacactgcgtacttcacagggtataatgcttcgattaaatactgtgtagttacctgattcagtgcttggcacgtaatagattcacaactgtttgctaattctaaattaggcaggcagagcatagaagtctgattaggaagattcattgctaggtagcaattagaaaaaaaatcacatggtagtgaattaaagcctaccaaatgttacagagatgaatataaacttgtattacatataactgcagagagatatagtttataggaaaaaaacgtgtaaagagtactgattctttggaagttttctctgaaagtgagggttgagtcagcacaatttgaatgaatattgttgaatggggaattgctattaagttagatttggttgcctctaggaaaagagacttagggccatgtaaagatgatatttggcaatgctggtaaactggttaattgccagaaagtcttgttgtttggtggggtttttgactggatgtaataaagaatctctctcataaggcttttggtggagaatgtagtaagacacaagtcctgttgaggaatattgttcttgctagtgtgtgtaggcatggaaagctggtatagtgaggaagacttgggtggttgaggacctatgctaaacaggaggtgaccggaagaaatggtaaaagaacttagcaccatgcctggctgtgaacaaggggagtccaagaaaactaagtgtccaaaataacatataagtttataatcttagagctagagaaaaattaggaaatagtggattattatgtttttaattgaagtgtaacatacatacagaaaactatacaaagcaaatgtatggctccaagaattatcaaatgaacaaatgtgtaaccagcaccccagtaaaaaaaaaaaagtatttgtcagcaccccagaaacccatatcattttccctcacgatcatagctcctgtttcccacaaggtaacagcgatgctaacttctggtattacagtttagttttacctgtttttttattttatataaactagatggtatgttgctggcttcttttcattcaacattgtatttgtgagaaccatccatatttttacatgttgtggctcttcattttctttgctgtgtagtagttaattgtatgaatatatcacaaatatttattaagtccactaacccaaatagtagttggatatttgggttgttttcaatttggggctattataggtgatgctgtagtgaacatttctgtacgtgtcttttagtgccctggtacatgcttatcttagtttgctcaggctgctataacaaaataccataaactgggtggctcataaacagaaatttatttctcaggtttctggatgatgggaagtccaagataaaggtaccagcatggtcaggttctggtgaaggccctcctcctggttgtagactgctgatttctcctcacatggtgaaaggagcaatcaagctcccttaggccttttttataaagtttccattcctgagtgtttcaccctcatgacctaatcacctcccaaaggtcttacctcttaataccgtcaccttggaggttaggatttcagcatatgaattttgaggagacataaacattcaaaccacagcaatgtttttctattgggtttacacataaagtttgggattgcttggtcgtagggtattcttgtgttcaatttcagcatattgtttacaaatagttttccaaagttattccaagttatattccagtatgttatagaactttccattgccccacatttttaccaacgcttggcattgtcagacttcttaatttgtaaccattttggtaggtgtgtagtgttaccaaattgtagtttagatttctttttccttgacttaatgaaggcaagttcatgtttactgaccatttggatatcctcttttgtgagttactggctgagtatcttgtcagggtttttttctgagttgtctgtctttttcttacttgaaaatatcttctcccaatttgtgcctttcttctttattctttttttttttttttgagacagagttgtcacccaggctggagtgcagtggtgtgatcttggctcactgcaacctccacctcccaggttcaagcagttctcatgcctcagcctcctaagtagctggaattacaggcacattccatcatacccagctatttttgtatttttagtagagatggggtttcaccatgttgcccaggctagtctcaaacccctgacctcaagtaatctgccctcctcggcctcctaaagtgattggaatacaggcatgagctgccatgccagcccttctttactctcttaatagtgatttttggtgaataaaaagttattttaatgtagttcagtttatctattatgggtagtattatcgtgtcctgtttaagaaatctttccctatcccaagataatgaagctattcctcttgtactaccttctagaaactttattgttctatatgtaatatgaagtaaagatcaaatttagactctatactttatttggattcactagcttttctaccaatgtgctttttctgttctaagatctaatccaggataccacattgcatttagacactctaccttttgaaactttattttggtccaagattttaagcttgtcactagtaatactagattatcatacatcactgcatgtcccacttctgctcattcaagggccttacgttgctgtctgtttgaactagcttcttggtaccttgatctggaaataatcttctcttcctctgcatttctatagattttctttttctttccctctctcatgctttattggagtacttttgctgatttgtctgtcctttctatgtgatagataaaatcaggcctggtacatgtttggctaagtgagacctgagccctacatgaaactaagtcagatcctcttaagtgtagtctacactgttttgttaagatgataaggtgacactgggttgatgacttgatccaacctaacgtggttggagaattaaaactatagaattaagttagcctagttgttttcaatcattctgcttcacaagaagttaaaagactagaggtatttgttgaatcctcactcattgtctctctcagcttcacagattgatactgtgctcctacagttgtaactccaagaaacacatttgtctttttagtacttacagctgtgaagctaaaggcaaatttgaataatttctttaaatgagtgtatttaaaacattgacttttctatgaatgatctcgtattttctgctctgtttatgcgtttatattttacaacatacagattatgtcttaggtctccttaattatacctccaaaccgctagtaagtagcaggtgcaaaattgaggaattgagggaagaactttgaatgcatgttatatgggaattgtatacttatacaatatgtagaagtagcagttatttatatagcaagctttgtttatttttttaagagaagattgcctccagatgaataagcagtaaatctttcatttatgtgaagtaagttatgttttttaaaactgtcgaatagtttgttgtttgaacataattctataagatattatataggatagtattctaagagaaataaaagcatattttcagtaaaagacttgtacacagatgtttatagcagtcttactcatactagcaagaaatggaagcaacccaaatgcccatcttctggtgactagttataaaattatgatatattcaaacaatggactaccactgaacaatgaatagcaatgaactactgataaatgcaataacatggatgaatttctaaaacatgatgctaagtgaaagaagtcagataggaagagtatatactgtgtacttgctgttatttgaaattgcacaggaaaaaccaaccaacagtgtaataagattagtggttgcctaggaccagggtgggttgattgcttgactgacaaggggcacagggaactttggacgaggggttggtagaaatgttctatatcttgattattgtggttacacaggtatatacatttatcaaaactcatcacttaagatagatgcatttcattatacttaacttatacctcaaaagaagttaccttaaaagtttaagactgggcacagtaacccatcagcatttggggaagacccggtgagaggatcacttgagcccaggagttcaagataagcctgggcaacatagggagaccccatgtctacaaaaaaataaaaactaaacttaaaaaaggttaaaaagataaaaaacagtttgtgacttagaaaactgatgctaagagaaaaagggtctgagatcacaggttgaaacagagggatatatgggaccaaaagcaatgaatttggtcagggcagacctaattgcaatgataaactttgagactttcacatatgattaaacaaattgtgtaatctgatagtaaagccttttgtattgagtatgaaaattgaaactataatttaattcttttaaaaattatccattatatacaaggagaaatcctgtaaaagtctgaaggaaagcaagcacaactggagtctaactggttgttgaagtgctattagatctagttctgggaagttatgtggttatgtagagctatagagtttttggaagttatgtagttatgtcccaaggctttgtcctctggcattgaggaaaactttagtacttgttttaaattgatagtttttaatgtagtcattatgtatatgtatatatacatgctgctctaaagacacatgcacacatatgtttattgtggcactattcacaatagcaaagacttggaaccaacccaaatgtccatcaatgatagaatggattaagaaaatgtggcacatatacaccatggaatactatgcagccataaaaaaggacaagttcatgtcctttgtagggacatggatgaagctggaaaccatcattctcagcaaactatcgcaaggacagaaaaccaaacactgcatgttctcacttataggtgggaattgaacaatgagaacacttggacacagggtggggaacatcacacaatcacacactggggcctgtcgtggggtagggggagaggggagggatagcattaggagatatacctaatgtaaaggacgagttaatgggtgcagcacaccaacatggcacatgtatacatatgtaacaaactggcacgttgtgcacatgtaccctagaacttcaagtataattaaaaaaaagaaaaaagaaaaatctgggatggctggctttagtttatactcagctgtgttacattaactctctcaaaacaaaatgcggtagataactaggtcaataaatgtgatcattagttaaaatgtgaaaatgataaaattttctagaaaaataaataccaaaatcaactcaaaaagatctagataacctatattcattcgagacagtgaattagtaatccgaaatcctcctttctccctcttttccctaccagagtatactaaaacctagaaagtttgctgcaaagtttcactgtgccttcacagaacagattatccctgtattgtacagcttatttcaggcaatagaaaaagagaaaactaaataactattttatgagagtgatagcaaaagtggacatgaacaataccaaaaaaaattttttaagggaaattactgtctcagtgaatacagtgaaaaaatactaaatgaatagaattttgtagtgtgtacatattaatgtaattctctgtattaaaggattaaaagattaaaggaacaaaaacactatgattgttttaatagatgacattaacattttttgataaattttataattaaccaaaaggagagagacctcttagcaaatttggattaaaaggaatctaggctgggcatggtggctcacatctgtaatctcaacatttagggaggccgaggcaggtggatcacttgaggcaggaggtcaagaccagactggccaacatggtgataccccaactctactaaaaatagaaaaattagccaggtgtggtggtgtgcgcctgtaatcccagccactccagaggctgaggcaggagaattgcttgaacccgagaggtggaggttgcagtgagctgaggtcgcaccactgtactccagcctgggtgacaaagcgagactgtctcaaacaaacaaacaaaaaaatctgaaatttcttttacctaataaagagaatataacaaaaacctagagtgagcaatcatgtttaatgataaaactttagaagcccttccattaaaatcagaaaaacgttaggaatgtgtgctagccctgcttctattaaacaatatgctagagggcttaggcactggaataacatgagaagaaattaaaagttaaaagaagagaaaaaattggtagtgagaataaaccatttatgttttgtaggaaattcttgtcaagaatggctctactgctccaattctagagttaatgtaaaacttaagtttaaaaaagccaggttcgggaacaggcaacctacaaaatgggagaaaattttcgcaacctactcatctgacaaagggctaatatccacaatctacaatgaactcaaacaaatttacaagaaaaaaacaaacaaccccatcaaaaagtgggtgaaggacatgaacagacacttctcaaaaaaagacatttatgcagccaaaaaacacatgaaaaaatgctcatcatcactggccatcagagaaatgcaaatcaaaaccacaatgagataccatctcacaccagttagaatggcaatcattaaaaagtcaggaaacaacaggtgctggagaggatgtggagaaataggaacacttttacactgttggtgggactgtaaactagttcaaccattgtggaagtcagtgtggcgactcctcagggatctagaactggaaataccatttgacccagccatcccattactgggtatatacccaaaggactataaatcatgctgctataaagacacatgcacccgtatgtttattgcggcattattcacaatagcaaagacttggaaccaacccaaatgtccaacaatgatagactggattaagaaaatgtggcacatatacaccatggaatactatgcagccataaaaaaggatgagttcatgtcctttgtagggacatggatgaaactggaaatcatcattctcagtaaactatcgcaagaacaaaaaaccaaacaccgcgtattctcactcataggtgggaactgaacaatgagatcacatggacacaggaaggggaatatcacactctggggactgttgtggggtggtgggaggcgggagggatagcatcgggagatatacctaatgctagatgacgagttagtgggtgcagtgcaccagcatggcacatgtatacatatgtaactaacctgcacaatgtgcacatgtaccctaaaacttaaaagtataataaaaaaaaaatatatatatataaaaataaaaaataaaataaataaaaaagccaggttcagttatagttgatgttgtctctatctctctgagcctagtaataataaaacactgttggttctgggatagtggaagaacttccttttcatttagcagttatattcataggttgtgcttaaactgattgtaattaaactgatgaaattatccaactaccaccaagtagttgtatagattttaaggatatctgtgagggaaaaaaatggtctattccaattattgaactactgttttatgtaaaaataatatgaaataaaagtggtatgaaatagaaaatggatggaaggatttttttgtggtaataatatctcttaaacttatattctgatttagggttgccttagtctgcatttaaacctgttcacatgctggatccaatcccagggccttaaagtacaaactgcttagccgaacttagtcttagctttaaaagccgaggtaacattgcagacccatggtgtattttagtcttagtcattatttactggtagcctggacagagtgcatggcatgtgctgttctgtgtcattcactctccttcacttcctccctacaatcctattttataatcagtttttacattttattgtttgtttatctttcctcttaggaagctgggattttctttttgctgaatggattgaaaaataattggggaaaaggaaaccacaaagagtttagagaggtttctgttaagtacaaaaattaacatttgagttaaattgtcttcgaattattttcacattatttatatatttaaaatgttttggctttgctcataaattcttcattgttcaaaacattgcttttgtaaaatttgtagtattccctttcaccttatctatcctgtatctattattatttttccctctttcagctttttgatgagaccacaaaggataatacttagaggagtttcctggcctgtattacaagatagaccatgagttctgcctcaattcaacttcattgtgtcaacttgataggataagacaggtggacattctgctaaccagcatctgattagagagggtggaggctggtgatggattgttaggtgtgatgacaaaataagcaattccgttaacatgagtgtgcagagtaaaattgggaccagcagatggtggggctaagctgtatcttatttctcagctatgagattttccgtggccgccttttcacagtagccagctgggattgtccattaactgggtttgagtaaaagggagttgttgctttctttagaatttgttcagcctctccttttcatgtatggctttatgttcatttggtagtaaaacacgatattcaaaggcagaatatatgagaactgaccttttcttggagaacatcccagttagatcccatttccacaatatgattacactttgaaatctggcttttccctgttctttctttaatcctctgatattttaaattcctgtaatctctgctattgccactttaaacctcattactgaaagttcttcccacactgaaacacttctcagaaaaaaaatgcagaatatagagcagagctataatataaacttaaacagacctgctagttttagctttcttttctagtatacataatttagtttacttgatccaaaggatctttaagaaacatgttttggtttaatttctgtttgttttgtttttttttttgagacagggtctcactgtgtcacccgggctggagtgcagtggcgtgatcttggctcactgcaacctccacctccagggttcaagtgattctcctgcctcagcctcctgagtagctgggacgacaggagtgtgccaccacacccagctaatttctttgtatttttagtagagatggggtttcgtcatgttggccgggctggtctcgaacttctggcctcaagtgatctacctgcctcagcctcccaaagagctgggattacaggcgggagccaccacgaccggcctggtttaatttctaaaacttacctactaatcgacttagttctgcaataaatatagttacaatcattataactagtattccttgggctggtttaaagatgttctttagcatttgagatgaaaggcagaaaccacaggtaggatcatgtaagctatggaaccaaaggaaaagcctggaaatgcaacttggagtcctgcttactctgtatccttggaaaatccagattgtgaaagaaaagaaaaagatcattttcatccatcttttgacagctttctactttgacacttctttcctctacagttccaacagaaagcccaaggctgactttgatttgcctgacttgggtatgttcccatccctgcctcaatcattaacttactggcctgagtcttagtgatggggtcagcctctcctcaatcctatgagcttggaacaggaaaggaaaattggagaagaggaaagggattctggacagtcaaaaataattaaatatccactctcttcccaaagctgtgtaatgggagagcactgtccttcagccaataatgcactagcagctagattccttagctagaccttcttccactgttgaagcctaatccctctgttttgctgcagatacctgtttccgaagtttacactgtgctggactgagtttgtagacatgaaggtccatgtaccctgtgaaaccctcgaatacattgaagccaactatggtaagacctggaagattcctgtaaagacgtgggactggaagcgctctcctcccaatgtgcaacccaatggaatctggcctatttctgagtgggatgaggttatccagttatattgagatagtaggttgaaatgggagaatttctcttttggaaaaaaaggtagataactgtttaaaaaatacatgtctatttgtcaaacataagtgggaaccaaagaaaaaatgtgacaagtttgaagacacagaaagagtcatctgatgtaattctctcacttagtactgaggaattttcatgtgccacatacaatgctaggttacagtggagaagcctagatgaatgagacaaatacctacttcttttattcctccttttggtaaacaactcaattttcctttgagggaaccctcccccaccctttgaagagttcaagttctgtacaggtttttaaaacgtgaagtaatgtttgaactggaagatgagctcaccaggcaaagctaaggaaggatatactagttgaaaagaataacccactcctcttctgggcatttaagctggtatgttagtgctacttttaagattgtggagtctgagttaatattcaagtgatcagactttgagtgacatcaagaaaagatgatatcaggttcatttttcaactaatcttatgtggaattgaattagagaacaaggcattattcttttagggaaggtgagagcttatttgtatcagagcttattacttgtcaggataagtaaatttctgtacatgtactgttttcatatgtgaagtgagaagaaactttatgcttgtttaatgcttaaatttccatccattgtgagaatattttcactgacctctgatggcacttgttgacaaatcattcaagtgagaccatgttactagacatgatcttgaaagaggccatgatttcacaaaactcatttttattttattctcagacagtctgttaggtaaaaatatgagaaattcatgtacattttatattttctgaatttataatctgtgcactcccaattttaatgacactaaaatattaatagaattttttaaatatactctaatttttaaaacatactctttattatcttcatttatcaattacagcttcgtatctctaatttatggtctatataccaatttaaatggcatgtaaacctgcctgtttcttctcctcttctaatatatcagatctccaaaatggaagctaaatggtggacttgacaactgttcaccctacctcagatcatagagtttgtaaagtttgtgtccctccccagtttttcagtctgttgaatgtcgatggggcaagaactcagacttctactttaccaagtaccacacactctggaatgctttagtttccttttcccctcaagatgtctgagtcagctaggatgctgtttaccccatctctctcttatatcacttgaatgatatattgtaagtgagaggtaaaggaaaatgtaggcacaataagcactgctatttttctctttgtctaggaaaggaagctgaatcttatatcttatctatgctatttaggactactttctggagcttggcagattttcctctgacaccagagaacaatagtagtctcaagaatggaaacctgaatgtctgagggaatgggctggtagactttttcgaaaacaaattagagaaagtaacttacaaccacccattccggatttgtaaagcaacatgaaaacctttgataaatgataaccaacagtcttctgtcctaatttgcattctcaatgcagaattattgggtctttcataaataacatgagtggtttctggagacatttaagattgtcagcaaacttgtcccaaaatggcacatcatcataatccattttctctttgctagaaaatcagcccatagagtgcattcccaaattctaaatagctgaccctaaattcatttttcatgcttaaaaataatagaacaaataataatactatttttgggcaaaatccaccctacttgatgaggaccatttgcttgtgctcagtatttagaaatgcatacactccacatttctccccatttccaattgggactcccattctttgccaggagatcttacccatcccttttcagattaatcttttatcctttcctgaagtacaaagtcttaagagtgtctgaaatccaagacatcttggcccaattgacacaggttctatattcttccctacatagaccactggctgctgaaatacttttcttgtcttctggtttcacaggcttcagctcatgggttccaccctaacttggggaaacaaaagccttctctagaatctgaaggccaggcttacctctgattctgattcatccatacttcatcttatgtattttaacagctgggttctgtggagtgtccagagaccttgggttaggtatatccatcttcagtacctcattggatcacttttctttcatcacttgagtattctagcagtcattctcctaatctgaccactttcaggtttagtttacctggcttacctggggaagttgacaacttgttggtagttaggcacccatgaatgtctccagagacatcctgagaggcaagattcctcttaattgataaccaggacaaccaggtagtcacccagtcctctctaagcagggagcacttgtccttctctcctctgctgcagctactgatatctggcccctggaataaaaccatagttcctaaaattgagcatccctaagagtagctgcttggtgggacagctgatttctttgattccctagctgcaaaacctgaaattgaccactaggtgacagaatgtttgccagtatccccacaaaacaagttaaaacttaagtgaaaatcattctgcttttgaatcttaaaagctagaaaaaccataatgtaatattctttttaaaccctcttattttataactaaataaataatcacagaaaagaatgatctgaacaagaacagctgaggctaaaacccaagactgccgtgactcctagtccaatgtctgtttcgcatcacaacacagtatctttaacagtgcttgagatgcttaacagagaaggcatccagtgcttcattgaggctaagtctcagggtgtttctgccgcttagtatctttttgttcagattgagaacctaaggcgacagagaggtcaaggggaagtattttctagttcagaattcagaattcttaggcaaccttcatacctttatctggaaaatgccttctctccagacaataagacagttcacatctggagacatcagcctttggtacctaattctctaagctcaagatgcatcccattgccactttaccattctatttcccaagggaaccatcagcaccaacctgctaaatgcctgtatttgaagtctctccccttcctgaagtgaccttttatgaggctctttccttcctaagggacctttccctggtagtagtggtctcattcacaaaaaagaataatagatgtaactggagtcactttgcagttttcaagattttttttttatctgcttggctggaaaggagactagagtatctagtttttagtatttaaactacttttaattatttatattgatactctctgataaatgcaggtagttaagaatagattgtactcattcctttttgagtttgtgacctcaaaccattgtttttattcttacacgactacagtacttcaaatggcacatagataggcaggatattacataggtaagcaggaatttatacattgggtaccagagctaaatctggaaaacacatttggaatgagcttccacacttcagtctaaaatctcacccaaacttatggctacatatttttctaagtttcccccctagtttcactttctggaaagtgaacagttttttaaatcctaaatgttataaatccttaggagaaatattccctcaaaacctagtcaagaaagtgccacattcccaccttctaacaggtaattattagttgtaatagctttaatgcatggaaaaacttcagttactgaccagtcaagagaatttctcaagaaaaatcccagcaacgttccctctttcctccttgtcttccactatcattaagacctgggctagatcacctctaacatctcactcagggaaggcaatgtgttgccataaaaagaccacaagcttttgagttaggcctgaatttgaatttcagcttaatcatgtgggatttatggtgggggccctttcagtctcaatttccacattagtgaactggggaaatgatacatacttctaagggtttttagggggattaaatgaagtatacagttcttagcctcaggcctaggattaagtaagtactcaagaaatgtgcaattttctagttccatgtttcttttctaatcttcaaatggaattatagaaaccatgggtcagaacatattcctttactcaaaagattgcatgactgaatttgcttaagaaaaaaaaaattgtgtctctccctctccctctccctctccctctccctctccctctccctctccctctccctctccctctccctctccctctccctctccctctccctctccctctccctctccctctccctctccctctccctctccctctccctctccctctccctctccctctccctctccctctccctctccctctccctctccctctccctctccctctccctctccctccactgtctccctctccctctccctctccctccacagtctccttccacggtctccctctgatgccgagccaaggctggacggtgctgctgccatctcggctcactgcagcctccctgcctgattctcctgcctcagcctgctacgcctcactggttttcgttttttttttggtggagacggggttttgctgtgttggccgggctggtctccagctcctagccacgagtgatccgccagcctcggcctcccggggtgccgggattgcggacggagtctcattcactcagtgctcagtggtgcccaggctggagtgcagtggcgtgatctcggctcgctacagcctccacctcccagccgcctgccttggccccccaaagtgccgagattgcagcctctgcccagccgccaccccgtctgggaagtgaggagcgtctctgcttggccacccatcgtctgggatatgaggagcctctctgcctggctgcccagtctggaaagtgaggagcgtctctgcccggccgccatcccatctaggaagcgaggagcgcctcttccccgccgccttcccatctaggaagtgaggagcgtctctgcccggccgcccatcgtctgagatgtggggagcacctctgccccgccgccctgtctgggatgtgaggagcgcctctgctggccgcaaccctgtctgggaggtgaggagcgtctctgcccggccgccccgtctgagaagtgaggaaaccctctgcctggcaaccgccccgtctgagaagtgaggagcccctccgtccggcagccaccccgtctgggaagtgaggagcgtctccgcccggcagccaccccgtccgggagggaggtggggggggtcggccccccgcccggccagccgccccgtccgggaggtgaggggcgcctctgcccggccgcccctactgggaagtgaggagcccctctgcctggccagtcgccccgtccaggagggaggtgggggggtcagccccccgcccggccagccgcccagtccgggaggtgaggggcgcctctgcccggccgcccctactgggaagtgaggagcccctctgcccggccagccgccccgtccaggaggggggagggggggtcagccccctgcccggccagccgccccgtccgggagggaggtggtgggggtcagccccccgcccggccagccgccccgtccgggaggtgaggggtgcctctgcccggccgcccctactgggaagtgaggagcccctctgcccggccagccgccccgtctgggagggaggtgggggggtcagccccccgcccggccggccgccccgtccgggaggtgaggggcgcctctgcccggccgcccctactgggaagtgaggacccctctgcccagccagccgccccgtccgggagggaggtgggggggtcagccccccgcccggccagccgcccagtccgggagggaggtggggggatcagccccccgcccggccagccgccccgtccgggagggaggtgggggggtcagccccccgtccggccagccgccccatccgggagggaggtggggggtcagccccccgcctggccagccgccccgtctgggagggaggtggggggatcagccccccgcctggccagccgccccgtccgggaggtgaggggcgcctctgcccggccgcccctactgggaagtgaggagcccctctgcccggccagccgccccatccgggagggaggtgggggggtcagccccccgcctggccagccgccccatccgggagggaggtgggggggtcagccccccgcccggccagccgccccgtccgggagggaggtggggggggtcagccccccgcccgaccagccgccccgtccgggagggaggtggggggatcagccccccgcctggccagccgccccgtccgggaggtgaggggcgcctctgcccggccgcccctactgggaagtgaggagcccctctgcccggccagccgccccgtccgggagggaggcgggcggggggggtcggccagccgccctgtccgggagggaggtgggggggtcagccccccgcccggccggccgccccgtccgggaggtgaggggcgcctctgcccggccgcccctactgggaagtgaggagcccctctgcctggccagccgccctgtccgggaggatggtgggggggtcagccccccgcccggccagccgccccatccgggaggtgaggggcgcttctgcccagccgcccctactgggaagtgaggagcccctctgcccggccacgaccccgtctgggaggtgtgcccagcggctcattggggatgggccatgatgacaatggcggttttgtggaatagaaaggcgggaagggtggggaaaaaattgagaaatcagatggttgccgggtctgtgtggatagaagtagacatgggagacttttcattttgttctgtactaagaaaaattcttctgccttgggatcctgttgatctgtgaccttatccccaaccctgtgctctctgaaacatgtgctgtgtccactcagggttaaatggattaagggcggtgcaagatgtgctttgttaaacagatgcttgaaggcagcatgctggttaagagtcatcaccactccctaatcttaagtacccagggacacaaacactgcggaaggccacagggtcctctgcctaggaaaaccagagacctttgttcacttgtttatctgctgaccttccctccactattgtcctatgaccctgccaaatccccctctgcgagaaacacccaagaatgatcaataaaaaaaaaaaaaaaaaaaaaaaaatcaagtcattaatacaattatacattaattatattacattaatacaatatatggtttgtgaattcagagacattaccagtttgcctccttctctcaatagaacttgtattttcattttcttggttaagcagttgtctcctaatattatcccatatgctacctagtttgctggtcccaagcagtttactgtacttcactagatttggtacctgctctcccctggacttctttttcaatattctagcctttcctagatgtaaatctttacctccttgttagtgaaattagatataagccatgatttggagagggaagaaatctggaatacttaatttcatttaattatctatgctgatgaatgcctgtatcattgttaataaaggagaattgaaaatactcatttctactttctgccctcaaatttctgtttctatctcaactaggcaagaatcagcagggtgcatgatgccattttaagctgcttcacatcagactgaaatcctaattacagttcataagtgaaacagactaattcaatggcaataccttttgtataggtcctgtgcttaaaggaggcaagtataaattttctaataagaaatccctgcttcttttgggtgcagtggctcacacctgtaataccagcagtttgagaagctaaggcaggtggatcacttgaggccaggagttcgagaccagcctggccaacatagtgaaaccccgtctcttctaaaaatacaaaaaaattagctgggcatggtggtgcacgcctatagtcccagctacacaggaggctgaggcaggagaatcacttgaacccgggaagcagagtctgcagtgagccaagatcgcggcattgcacttcatcctgggcgatagagcaagactctgtctcagaaaaaaaaaaaaaggaaagaaagaaatctctgcttccgtactatcaaaacttctaccctagaataccccctggcaccttctaacccaacctaatacagagattttgtagggacccattaacaagctcctatataattataagcagctctcacagtagggttgaaagagaatataaggaaaattagaagtactgtatttttgctattggaaatgaaatattgtttcatgcacctttgaaaaaaataacaggattttacagccttctgatgattcattcaaagcatggggaatagttcatatgtttgttaaatgaaaatcttatgtagctatttgtgtgtccctcccacttcataactacaaaaacatatatatgaatttctaaacaaagtgatattttaaagatgaattgattcaatgtgtacttaccagtttactgtgtggttttatcttcaggtacagatagtttgtggtactacttgaaaatacctttaatattattttcatcagaatttgtaatatataatccagtttgggatgatgaataaaatttttctaatctcttgagatatcttgtatttatttttgagacttgcagtagaaataacagacactaacattcacagacaatctgataaaatagtaatcttgccaccagtacagtatttctaaaattcaactatggggaccctagtagtctgcacacatatacctgggtatccaaaagttctcagagataaaacctgccagccaaagaccaccaggaacacacctgtaatcaaacaaagttaggtttattagcttgttgtagtaagaggaaacagccaccatggggaatcataacatatttcagggagaaggaactagaaaggtcttttataggctttgagctgatgtcaaaattgttaaaagtaactgtggtggagtggaaataacacaggacatggagtaaaaagttctagtttgtctgaatccaacagtgccatgaccagtaggattcatttcaggtgtacatggctagttcagccttaaaacagtcaatgtaatgcactgtatcaacaaagtaaagaaaatcatatcaatagacacaaaaagagtctgacaaaatctaaccctcattcatgagaaaaactcagtaagttaaaaatagaagataattacctcaacttgatgaagaacatctaaaaccaacaaacaaaaacctgtatgttttaatagcaaaaaactgaatgtttttcctctaagattaggaacaaggcaaggatgtctgctttcatcactcttattcagcctaatactagaagtgctagtcactgaagtaaggcaaaaaataaataaataaataaataaataaaagacatgcagattgcaaagaaatttttaaaaacttttcatttgcagatgacatgattgtttacatagataataccaaggaatgtattttaaaacaagcaaacacctggagctaataagtgagttttagtgcagtcacagtatacaagatcaagaccaatacccccaaatcaattgcatttctatattctaacagcaaacatgagaacaaaaacacagtactatttaaagtcaccctgaagaaaatgaagtacttaggtataaaattaacaaattatatacaagatttgtatgttaaaaatgctgatgaaatcaaagacctcaataaatggagatgcataccatgttcatggattggaaaacaacacagtaaagatgtcagttctactcaacttgatcaataggtttaatgcaattcctatcaaaatctcagcaaggtttttaatagacatagacaaacttattttaaaatgtatgtgataagtttatttctctagaatatctcaagtaatctttataaggaaaaagtagcagaaagatttggtatcagaagacctaagttcattcttgcacttcaatagataccacatctgatcttataaggtagatgttatttccccttgttttgcagatgaggaagctgcaatttagaggtaacacagatcttaaatccttgttttctgacttgaaatccagtggctactcactctgccaattctacttaactgttgatctgaaaaaaaaaatttttttttaattattacttaaaaccagcctctgatactgaaagtgagaaggatcactctacccaatattaaggtttattatatagctatagtaattgttatgggctgaattgtgttcccttatatccctcaaaattcatatgtttcagtcctgacccctagtatctcagaatgtgactgtgtttggagatagagcctttaaacagctaattaaggtaaaatgaggtcatatgggtgattcccaattcactggtgactagagtccttagaagagcttaggacaaggagaggcacagaaggaggaccatgtagagacatagagagaagatggtcacctacaagccaaggagaggatccctcagaagaaaccagccctgccaacaccttagccttggacttctagtttcctgaattgtgagaaaatagatttctattgttgaaaccactcagctgtggtactttgttatagcagccctagcaatctaatgcagtagtcaagacagtatggtattggtaaaaggatacgcacatagatcagtgaaacaaaataaaccagaaattgacccatatgagtatgtccaactgattttttacaaaagtgcaaaagcaattcagtggaggaaagacagtctgtttttttttattttttcttttatagacagggtctcactgtgtcacccaggctggagtgctgtggcacaatcattgttcactatcacctcgagctccatgggctcaagcagtcctcccgcttcagcctcccaagtagccaggactacaggtgtatgccaccacaccccgctattattttattttattttgttgttgacacggagtctcattatgttgcctaggctgctctcaaactcctggccccaagctgtcctccacctaggcctcccaaagtgctgagattgcaggcatgagcctccacacccagccaagatagacctttcaacaaatggtgctagagcaattggacattcataggcaaaaacaaactcaacttgaatgaacctcacactttgtacaaaaatgtacttaaaatggatcacatgcttaaatgtaaaatataaaactgtaaacccttttgggaaaaaaataggagaaaatcttcatgatctagggttatgcaaagcattctttctttgacttgacacaaaaatcacaatgtataaaagaaaaatggataaattggacttcatcaaaattaaaaattgctgctctgcaaaagcccacatgtaggggctgaaaagtccagctacagactaggaggaaaatatttgcaaactgtgtatcttgacaaaggactagtacctggaatatataaagaacctgaacactcagcagttttttgaaaaattcaattagaaaatgggcaaagacatagacagacatttcattgaagaggatatacagatggctaagaagcacatgaaaaagatgttcaacatcattagccagggaaatgcaaattacaaccacatgagatatcattgcatacctattagaatggctaaaattaaaaataatgataacaccaaatctgctagttgtttcttttatgattttcttttttaatgtgtactgtgcaccgttgtttttactgtgattttactaaagagtgtccttaaacattttacaaacattcgtaataggtaacactcttcataataaaaaggaataaccttgtctgaatttttggaagacaggtttttaggtttttgtttttgcctttcctccaattctttgttgatttactttgtcattttaataaccctctttttatgatttattttctctttattattcctttgtgttcttcgagttttctttaattagatttatcagtaaagccctttagcagctagtactattgttcatagttctctgcaactttatcagtagggcttttacaacctaaaacttctaaattcaaattttttcttccgttaatctcaataatttggaggatgttttctagtgaattttgcaggaaagttaattgagtggccaatgttctgaaaatgctatactaccaaatgtctttcagatgacttagaagatgacagtctcatagttggagagtggaagagtttgctttggagcccaaactgggcaaccgtctaatccagccagatcctgcttagcagaaaaagcaaatttctggcatgtgacctcataaacaagggaaaagctctccttttaggatgatgtcttctcttaccatctatttccccatgtcttagtggaaggagccatctttttccccatgtcttagtggaagaccagagaattatctagagcatggtgtgatgctgcaaatgatgtatctgtagccactagccacatgactactgaatatttgaaatgtggcaagtgtaactgaataactaaatatttactctaattttaattaatttaaaactagtagctagcatattgcagatctatagggttttatgggatcagcaagggttttggatttgtcgactggaatccagagccctccacagcctagttcggtgatcttgggctagctattcaacttctgagttctgaattttttttcaactaatggggctaaattaatacctacctttaaaggttattaaaagaattgtaagaaattgtaagaaatctgcagtgtctggcacactgctcagtacatggtagatgtacagtacatggtagatggtcagtgaatgataactattgttaatattatgttcacatggttttacatctgcctttggcataaatcctatcagcttgtattttcctgataatctcatgtcacaatttttctgtaagattggtatttcagatccctcctgggtagaggccctatcctgagcactggtgttaagaagcgaccctggcctcaagagcacaggtacaaggcctgttctttggggagagagtatgtggggttaaaacataacacttaatggaattgagtctcaaggaccaggcttaggcaaagagacaaaagtcctagactttgtagatggctgtctgagcacccgagtctagaaaaagctccaggaaggaggacagggactgggtaatgaggttcagctgagtcttaggacttgtagaacagaaaatttgaataaatgaagaaagaaaacatttctgagtaagaggagtcagtaaattcacagaataggctttatgggacagtgaataagaccatctgccatatggataaatagtgaaagatacaactggaaaagtggtcaaggaacagactgcaggaaatgaggggactgaatattctgctatgaagtttggatatgagagagaaaagttttgaataggagcatcatgccttcaataaacacttctggcctggttactactcatcggatctgtcctaagggtgaggttcgacaaacattcaggaaaccccttcaaggatagagcagggatttaggagaattcagattcaccgagactgatcctagagaccctagaaccctgatagttgcagggacagaggatacaaacttagccagatgggcataggaccctagtggtttaagtaaggtcactcctaggaattatcagtcagtgctagacatgggcacaagcagtccagagtcaggaagcgcttgagaccaagtgagcaggggacagtttggtgatggtctgggaagtggagctcaagagcagcattgcaagccacagaaagggagtgtgataggacaaggcagggtcttatccagagggttccagggaattagaataggcctttgagagccatgacaaaagctcattttgatgaattgggccaggagagccagtgagattctaggctgtggagaagacatgaaggcaatttttggaagacagcagaggaatggagaccaatggtcagtgctagacctgggcaccacaatacaggcaatgtgagggatgtgggaaagaggctggagccatttctatacctgtcgcttcagttagaaactaggacaggatagacttttcacatgatgatgccacagggcataactgaaagctagggagaacagaagccaggaagggagataagcttagtgaggattttaaattctgggtcttaacttagtcctcatctccctattggctgttcacctctggagactatgggctccaaggcgtaaaaagtaattgctctagttgtactaggagagtagtttgtgctaacaactgaccttctaccctacatttacctctacgagaaggcttgggactccagtggctttctggaccataataaaaacaaggccattttgtcttcactcttcctcgtttccacccagacagattctgctgcctggataagacagctcaggcagggaccgctggctgacgaggcctgggcaagcctataatcccagcagagagcacagggacaatgagtgggaggggagccagtcacaggttgtatcttattaaaccagtctgcatcagctacagtgtacgtctcagaaacagatctgaaaccccagctggtaacctagttagttcaggcagcgtgtaaagaaaccatatccccgccagctaaaaagatgcatgtgctcctgggtagtgcagaagtatctgttatgaaaagcaaaggtaacaacagttgtgggaaattaaggtttcctctgtgtgtttttttattggttgcatttgaggtgacatcctctaattttcctaagcacagtggggcctcctggaaacatctgctggatttgaggagtaaggggatgcttccctcatcctccgggtgtgtgtatttggtttgggatttgtcaggctgggtagctgagggctctgggcagcttgacctggcagatttcccccacttgcctgaaaagcagcctagggggcagaggcccctccccaactcagccctgcaccttcactctaagcgcctggagctggggccttttatttcaagtctggtccccagggagcagagtgggaaatgaggacagctgataagcctgacagtattgactttatggggagtattcaatgaatttactttctgcaagtaggctgcactcttatctgctgcccacagagcatctaaatcctcatctaggagacccatcgatgagtcacgtcccttacacaaagaccagagaataaagaaggaaaggggaattccatccacccctttcttttctccagtacctggtcctgcccaccccaacacctcccctcgctttccccactgcgtttgggtttattggctgaaaacagaagcactcgcagctccaggcctacggagtcaaggccaagccagcctggtcttgagaggtcgacagctgggcacacccagggctgtatgtccctctaactggtaactatgggaagctcacttgaagtagttgtgtgcaccgctttatgctgcaacagtcaacatttgctctggacagaaataccctcacggctttaacgccaggtgtcttggagataaaatgtgggtgtgtgggcgttaccaaggggtcctgggtctggggtgctggagagtggaagttacatgtaagagaaaggcctgatgcgcaagagaagtttttctttcccctctggcttctccctcatccagtcctgggctctgtttcaaatattagaaaaaaataaaagcttcttagcagcacagaaagtaagtaacttgaaggagagaggtgggagccagaatgctggattgggcagatgaaaggaaaaaactgaaagtgccctttggcagaaattagagtcatgtgtttaggttcaccatctagcttttagacagagttttttggtagtaaaaataaaatgaaatctctgtattgagtaactttggtttcattagatgacttagcaccattttttagtatttattccaaagcactaactttttatacattagctcactgaatcttcacaataacccatgagatgatatttctgagttatagctgagaaaactgagtctgggataagttaagtaacttgctcaggatgacaactataatagcatcaaagcaaggatgcaaacaccagccagtctgcctccaaagccaagtcaaaggtcttctcttagctgccacactaaactgcctgctatttggcatttttcaatatcttatctcagtccatggccaatcaatgagtatttattattcccacgttattggaaacaggcttagcaggataccactacctgtccagggccacaaaaccagtgtatatcagagactctggtccacagagtctagcatctctcctaaaggtctcgccctgctggtgcattgcccactgctcaggcagagatgtgggccacatcagtgcgtttctcccttccaggtgccctggtttcctgtgtcacctgctttcacctgctgctacttgcttgataattttcttagttgagggaggttggaatgagggaggcaggaagagcctgggaggatgtgagctgttcactaagttgctctgtgggccctgtgaatggagtagtatgaacatccatgagaatctgcagcttctgcaggctctggaaagatgcctgtctaaaaaccgctagtaaaactgagtcagccatatgcttgtttctttaagtatatgttttagtatttgacttctttgggagaaatacattttttgtttaggataacttgttatgtaactttataattaatatttataattgttcatattgaataagaaaaccttggtgaaatgcctagcatgacacttggcacttaaggttgaataattggggcagaggattaagttcctgggccagagttgatgcttaatgtcaacccctcctcaggtcaagccatcatctcctcttgcctgcattgctttcacggcatcctaactagtccccccaccccacctcttctcttgcccctctccatgtagcagacagaatattctctccttcttaaaaaacaaccaggttgggcgccgtggctcacgcctgtaatcccagcactttgggaggccgaggcgggcagatcacgaggtcaggagatcgagaccatcctgactaacacggtgaaaacccatctctactaaaaatacaaaaaattagccgggcgtggtggcgggcgcctgtagtcccagctactcgggaggctgaggcaggagaatggtgtgaacctgggaggtggagcttgcagtgagccaagatcgcaccactgcactccagcctgggtgacagagtgagactccatcttaaaaaaaaaaaaaaaaaaaaaaaccattctatggccttggaaacatttacctcacagaagcaagctatgtgtctgctgacagaaggcagggcaggctggaggcagctgtctgaagaaataagagctttcttgcattcattcaacaaatatctgatcaagcagcttttatgggcagtgagcacaattcctggggtctagtgatgaaggaaactaagtctttgtcctcatgaagtttataatgtagcaagtaaactagaatgagatttgttttgcagaattcaacatgaaggtggggtctcctttaaagaaaaaaaagagagagttaaaataattgaaatttatcaaaaagagtttcttatgaccaagagtcactcccacgcaccccaaattaagtataaagaatgggcacagtttactttggaaaatgcaaatttaaaagcaggggttgtaatattaatataataaaatgaaattcatggtaaaaagcaagatttttatattgatataggctacaatcctctaagtcaataaaaaaacttccttgagtctttatgcttcaaaagcaatgcagcaaaaaatgtaaagatctaaagcaaacactcccggaaaaacaaaaagaacagaaacaaaatagtaaagggagattttcacacagtgctctcttgaatagatcaaatagacaaaaacttccaagaatacagatttatttaatggatgtgtaaaaagacattttaccattcaaacagagaatatacctccttttctagtacctgtgaaacatttataaaagttgaatatatgttttatcaaagagaaaattctcaataaatatcccaaagcaaaaaacatacagggcatatatttcactatactgcaataaaattagaaactaatagcaaatggttgccaaaaaaatacaacaacaagaaaatttaaaaacactttataaaagaaaaataagcaacagacattagaaaccaatgacaatgatactacaaatggaaacaggatatccccaaaggtctatcagaagaaagttcacagcccggagtgcttttcttactaaacaagaaagagtaaaaataaataagcattcaatccaagagtgatagagtggagaggaaataaacgtaaacaaaagaacagatttaataaagatatagtagaaagtgtatttgaaaatcataaaaatgataagcgaatcccagagctagttttttaggagcaataaaatgaacagacttttgcaacactgatcaagaagagagagagagaaatcataaacacataacatgaggcatgagaaaggggattaaaaaaatagagatgttaaaaagtaactgaataactgtatataacactctactaatgaatctgaaaaggtccaaatttatatgtcaaagtaccaacattaaggagagagagaacaggggaaggaacaaaacctacctagaaggatttactagtaaattgtattaaatatcaagaaccagctaactcatctgtttaataaattaatggtggatggaaaaagtgatgaataaatgactggataaatggagagatggatggatgaataggggcctcgatacatagaattggagattggtaaaggggctaaggatggaggagggaagaagagagttttaagagtggctaaggctgatgcttgacctccagccaaaacaatcttggcccacacccacttggcctggcagaaatcccttccaaaagtcccaggtttgggccctggcggtggctgactcctgtaatcccaacactttgggaagccaagtccggaggattgtttgaccccaagagttcaagatcagcttgggcaagatggcgagatcccgtctctacttttatgaataaaataaaaaacaaaaatcccaggtttggtctttcctgaaactgacaacccctgcatacaggactagaaggccagtattcacaggctaatccagacagatcaattaaaccaggagaaccagaaagcctgacagtgcccaagctctcctagtgacctgcccttccctccccagccctctgtttcctccccaggagctcgcaggtgcagtctctccagggggcagtgagagccatgaatagtaagggttttagctcaagcacacagaggcgtttagctgcccaaatctaatcccccaataatcggcttatgtaaattcctacttcaaccccttcccctgcaggtcctagccccaaaattctctacattgggagactggcatgggagaagacccatcactctgaaggatcactgctagtgaaatgatgcgccaaagattgtttcccctgcttctgaaagtataaaaccaacaataacatttaagaatgttttgaaaagaaaaaaccatcaaccctggtcccaggatgtcaacacaatcgggctcctttctctgtagcccttgtcctttctctgagtccttgtccactcgcacacagatcctatttgacagcttattgtttcgtttagcatcatccatttccaatcttgctaccctgttaccacaattctttttctcagctgtaaaatatgccattcaaaaaaatatatcaccttacagtttttggctgaggtgaagattaatacaggttattgcttcaaaatgtaacatttgctgtattataattgccatatggggaaaacagaggagcagaaagaggagcaaatcagagaagcttactgcaaatattagtttttgtagttgtttgtttttctagatggagtctctgttgcccaggttggagtgcagtggcatgatcttggctcactgcaacctctgcctcaagcgaagcgattctcatgcctcaacctcccaagtagctggaattacaggtgtgcgccaccacacctagctactttttgtatttttagtagagatggggtttcaccatgttggccaggttggtctcaagcccctgacctcaggtgatccacccacctcggcctcccaaagtactgagattacaagcatgagccaccgcacctggccttaggttatgtttctaaagatccctttttaccaactaattttccccaatccaccctccaatctctcctctatactgccaccagaatgagtcttgcgacctgtgactaaacatactattcccatgttcaaagcacacagttgtatttgtctgggctgccctctcctccacccttgcacttgtattataattcctacccagtctttaccacccttccaccaggcacccagcagtcagagcccctcccctggacactgtgcttttagatggcccctctctggccctcctccagtgctcacccaactcctatgtcccaccttctagaacatattctgggaacctgggacccctgaatttctgttcaaatgaccatgaacccttttccagggcctggatagggctattccctaggtccatgtgggctgggagttcgcatcattttcacaaggcccttcacagaaaaagacagagctagcgggtgggaaaagaatggggacggggatggagtctccatttgtacccttatcatggcccccacaaatgtcagagccacccttgcttcaaggcctagtttaaatgccatctgtcccatgggtaacctctgatcccccagctagaatcttctacctttctgtccctaactctaatttcacactctctcgcattcaggactgtctgtcttatattagtcatgttgtcatgtcttctcccttccaatagctgttagtgccttgaaaatagatacagagctttcctcaccttcatgcctacctccccatcctaccccactcccctcctaccaccataacctagcaatttatgcaacaccttttaaatttataataaaactgtattgtttgttttggaggtgggtaaggtgggtggcggtgtgacaaacaaccccaaagtctcagtgacttacaacaataaagatttatttctactcatgttatatggttggttgtggttttgctccatggcatccaggctgcacgagcaaccccaaacataactttctcatggctgagcccatccagcaatcccaactggagtcttgctctatccccaggctggagtgcagtgttgcaatctcggctcactgcaacccctgcttcccaagttcaagcgattctcctgcttcagcctcctgagtagctgggattacagtcgtgtgccaccatgcccggcaaatttttaatttttttttagtagagatggggttttactatgttggccaggctggtctcgaactcctgaactcaagtgatctgcccgccttggcgtcccaaagtgttgggattacaggcatgagccactgcagccggtccagcaatcccttgtaaagcttctgctccatcatgatcaatgttagggctgctcgcattctattggctgatgcaagttgtatggtcaagcctggcaatggggcagggaagtatagttcctccacttacagggaggcactgccaatcacacggcagtgagtggggctatataatcctctccaagggaagggagccaatagttattaacaataatacaatggaccacaataaaatttacaatataccgactatgtgctaggcatactgctaaatgctttacctacttttttctcatttagtcctgacaattctgtcattgtccccattttacagatagggactaaggcaagcataaattctataatttgcctaggatcacataagtgaatagacaaggaatttccacctgggtaatgtaactccagagccctttgctcttatccactaagctgcaatttgtttgtgaatttattgtgccaggtcctataccagatctttcagagagagtggtacctgggaattcattacttattcattcattaatcaacatctgatgaacacctgttcactgggagtagatggggtagggaagaggcagagaagataaataagtaaataatactcaagtggggatgagtgttaagaagaataaagcaaacagaaggatgaagactctgtgtgtgtgtgtgtgtgtgtgtgtgtgtgtgtgtgtgtgtgagcaattttagtttttttttttttaagagacaaggtttcactatgttgaccaggctggagtgttgtggctattcacaggtgcgatcatagtgcactgcagcctcagactcctggcctcaagctatcctcttgcctcagcctctggagtaggtgagattacaggctcactaccacgccagacagatggtgcaattttagatattgtggtcacagacttcactgagaaggtgccatttgagtaaagacctaaagaatgtcagctccttgagggcaaggacttgtatctgttttgtttgaagttgtgtccccagcaactagaacagggcctggctcattgtaagctctcagtaataatgtgttgaacgaatgaaaggaggttagggagggaatcgtggataacttgggggaagagtgtttaaggcccaggaaacagtcagtgaaaaggctctgaggaaggagagtatctggtgagttcctgaaacaacaaagagaccagagtggctagagctgagtgagccccaggaagagaagagacagacagctcagggggatagaaggtatctctgggcccattttaaaggcttcagcttaactcagtgaaatggagagccactgaggggttttgagcagagaagtgaccagaatctgacttgtgttttcatagcatcattctggatgatgttggagaacagacagaaggaggcaagtccagaagcaggaagaccaattaggagtcccttccctcactgaaataaccaatattagtgctgggcattgtggaaactgaaatggataaattcgggaacctgcccagtacagtgaatgttaaattctgctgtgcatcttaatctcctgaaatacttaggttttaaaaatgcagatttcagaccacaccccccatcctgaaaaatcctagtttcctgggtctgggttgtgggtgttgggatc